European Patent Application EP 4 324 518 A2, published February 21, 2024. Title: ANTIBODY MOLECULES TO TIM-3 AND USES THEREOF. Applicant: NOVARTIS AG. The sequence listing filed with the application follows.

SEQUENCE LISTING (142 sequences)

SEQ ID NO: 1 - protein, 118 aa, synthetic construct
  REGION 1..118: note = source = /note="Description of Artificial Sequence: Synthetic polypeptide"
QVQLQQPGAELVKPGASVKMSCKASGYTFTSYNMHWIKQTPGQGLEWIGDIYPGNGDTSYNQKFKGKATLTADKSSSTVYMQLSSLTSEDSAVYYCARVGGAFPMDYWGQGTSVTVSS

SEQ ID NO: 2 - protein, 111 aa, synthetic construct
  REGION 1..111: note = source = /note="Description of Artificial Sequence: Synthetic polypeptide"
DIVLTQSPASLAVSLGQRATISCRASESVEYYGTSLMQWYQQKPGQPPKLLIYAASNVESGVPARFSGSGSGTDFSLNIHPVEEDDIAIYFCQQSRKDPSTFGGGTKLEIK

SEQ ID NO: 3 - protein, 5 aa, synthetic construct
  REGION 1..5: note = source = /note="Description of Artificial Sequence: Synthetic peptide"
SYNMH

SEQ ID NO: 4 - protein, 17 aa, synthetic construct
  REGION 1..17: note = source = /note="Description of Artificial Sequence: Synthetic peptide"
DIYPGNGDTSYNQKFKG

SEQ ID NO: 5 - protein, 9 aa, synthetic construct
  REGION 1..9: note = source = /note="Description of Artificial Sequence: Synthetic peptide"
VGGAFPMDY

SEQ ID NO: 6 - protein, 15 aa, synthetic construct
  REGION 1..15: note = source = /note="Description of Artificial Sequence: Synthetic peptide"
RASESVEYYGTSLMQ

SEQ ID NO: 7 - protein, 7 aa, synthetic construct
  REGION 1..7: note = source = /note="Description of Artificial Sequence: Synthetic peptide"
AASNVES

SEQ ID NO: 8 - protein, 9 aa, synthetic construct
  REGION 1..9: note = source = /note="Description of Artificial Sequence: Synthetic peptide"
QQSRKDPST

SEQ ID NO: 9 - protein, 7 aa, synthetic construct
  REGION 1..7: note = source = /note="Description of Artificial Sequence: Synthetic peptide"
GYTFTSY

SEQ ID NO: 10 - protein, 6 aa, synthetic construct
  REGION 1..6: note = source = /note="Description of Artificial Sequence: Synthetic peptide"
YPGNGD

SEQ ID NO: 11 - DNA, 354 bp, synthetic construct
  misc_feature 1..354: note = Description of Artificial Sequence: Synthetic polynucleotide
  source 1..354: mol_type = other DNA
caggtgcaactgcagcagcctggggctgagctggtgaagcctggggcctcagtgaagatgtcctgcaaggcttctggctacacatttaccagttacaatatgcactggataaagcagacacctggacagggcctggaatggattggagatatttatccaggaaatggtgatacttcctacaatcagaaattcaaaggcaaggccacattgactgcagacaaatcctccagcacagtctacatgcagctcagcagcctgacatctgaggactctgcggtctattactgtgcaagagtggggggtgcctttcctatggactactggggtcaaggaacctcagtcaccgtctcctca

SEQ ID NO: 12 - protein, 11 aa, synthetic construct
  REGION 1..11: note = source = /note="Description of Artificial Sequence: Synthetic peptide"
SESVEYYGTSL

SEQ ID NO: 13 - skipped

SEQ ID NO: 14 - protein, 6 aa, synthetic construct
  REGION 1..6: note = source = /note="Description of Artificial Sequence: Synthetic peptide"
SRKDPS

SEQ ID NO: 15 - DNA, 333 bp, synthetic construct
  misc_feature 1..333: note = source = /note="Description of Artificial Sequence: Synthetic polynucleotide"
  source 1..333: mol_type = other DNA
gacattgtgctcacccaatctccagcttctttggctgtgtctctagggcagagagccaccatctcctgcagagccagtgaaagtgttgaatattatggcacaagtttaatgcagtggtaccaacagaaaccaggacagccacccaaactcctcatctatgctgcatccaacgtagaatctggggtccctgccaggtttagtggcagtgggtctgggacagacttcagcctcaacatccatcctgtggaggaggatgatattgcaatatatttctgtcagcaaagtaggaaggatccttcgacgttcggtggaggcaccaagctggagatcaaa

SEQ ID NO: 16 - protein, 118 aa, synthetic construct
  REGION 1..118: note = source = /note="Description of Artificial Sequence: Synthetic polypeptide"
QVQLVQSGAEVKKPGASVKVSCKASGYTFTSYNMHWVRQAPGQGLEWIGDIYPGNGDTSYNQKFKGRATMTADKSTSTVYMELSSLRSEDTAVYYCARVGGAFPMDYWGQGTLVTVSS

SEQ ID NO: 17 - DNA, 354 bp, synthetic construct
  misc_feature 1..354: note = source = /note="Description of Artificial Sequence: Synthetic polynucleotide"
  source 1..354: mol_type = other DNA
caggtgcagctggtgcagtcaggcgccgaagtgaagaaacccggcgctagtgtgaaagtctcttgtaaagctagtggctacaccttcactagctataatatgcactgggttcgccaggccccagggcagggcctcgagtggatcggcgatatctaccccgggaacggcgacactagttataatcagaagtttaagggtagagctactatgaccgccgataagtctactagcaccgtctatatggaactgagttccctgaggtctgaggacaccgccgtctactactgcgctagagtgggcggagccttccctatggactactggggtcaaggcaccctggtcaccgtgtctagc

SEQ ID NO: 18 - protein, 444 aa, synthetic construct
  REGION 1..444: note = source = /note="Description of Artificial Sequence: Synthetic polypeptide"
QVQLVQSGAEVKKPGASVKVSCKASGYTFTSYNMHWVRQAPGQGLEWIGDIYPGNGDTSYNQKFKGRATMTADKSTSTVYMELSSLRSEDTAVYYCARVGGAFPMDYWGQGTLVTVSSASTKGPSVFPLAPCSRSTSESTAALGCLVKDYFPEPVTVSWNSGALTSGVHTFPAVLQSSGLYSLSSVVTVPSSSLGTKTYTCNVDHKPSNTKVDKRVESKYGPPCPPCPAPEFLGGPSVFLFPPKPKDTLMISRTPEVTCVVVDVSQEDPEVQFNWYVDGVEVHNAKTKPREEQFNSTYRVVSVLTVLHQDWLNGKEYKCKVSNKGLPSSIEKTISKAKGQPREPQVYTLPPSQEEMTKNQVSLTCLVKGFYPSDIAVEWESNGQPENNYKTTPPVLDSDGSFFLYSRLTVDKSRWQEGNVFSCSVMHEALHNHYTQKSLSLSLG

SEQ ID NO: 19 - DNA, 1332 bp, synthetic construct
  misc_feature 1..1332: note = source = /note="Description of Artificial Sequence: Synthetic polynucleotide"
  source 1..1332: mol_type = other DNA
caggtgcagctggtgcagtcaggcgccgaagtgaagaaacccggcgctagtgtgaaagtctcttgtaaagctagtggctacaccttcactagctataatatgcactgggttcgccaggccccagggcagggcctcgagtggatcggcgatatctaccccgggaacggcgacactagttataatcagaagtttaagggtagagctactatgaccgccgataagtctactagcaccgtctatatggaactgagttccctgaggtctgaggacaccgccgtctactactgcgctagagtgggcggagccttccctatggactactggggtcaaggcaccctggtcaccgtgtctagcgctagcactaagggcccgtccgtgttccccctggcaccttgtagccggagcactagcgaatccaccgctgccctcggctgcctggtcaaggattacttcccggagcccgtgaccgtgtcctggaacagcggagccctgacctccggagtgcacaccttccccgctgtgctgcagagctccgggctgtactcgctgtcgtcggtggtcacggtgccttcatctagcctgggtaccaagacctacacttgcaacgtggaccacaagccttccaacactaaggtggacaagcgcgtcgaatcgaagtacggcccaccgtgcccgccttgtcccgcgccggagttcctcggcggtccctcggtctttctgttcccaccgaagcccaaggacactttgatgatttcccgcacccctgaagtgacatgcgtggtcgtggacgtgtcacaggaagatccggaggtgcagttcaattggtacgtggatggcgtcgaggtgcacaacgccaaaaccaagccgagggaggagcagttcaactccacttaccgcgtcgtgtccgtgctgacggtgctgcatcaggactggctgaacgggaaggagtacaagtgcaaagtgtccaacaagggacttcctagctcaatcgaaaagaccatctcgaaagccaagggacagccccgggaaccccaagtgtataccctgccaccgagccaggaagaaatgactaagaaccaagtctcattgacttgccttgtgaagggcttctacccatcggatatcgccgtggaatgggagtccaacggccagccggaaaacaactacaagaccacccctccggtgctggactcagacggatccttcttcctctactcgcggctgaccgtggataagagcagatggcaggagggaaatgtgttcagctgttctgtgatgcatgaagccctgcacaaccactacactcagaagtccctgtccctctccctggga

SEQ ID NO: 20 - protein, 111 aa, synthetic construct
  REGION 1..111: note = source = /note="Description of Artificial Sequence: Synthetic polypeptide"
DIVLTQSPDSLAVSLGERATINCRASESVEYYGTSLMQWYQQKPGQPPKLLIYAASNVESGVPDRFSGSGSGTDFTLTISSLQAEDVAVYYCQQSRKDPSTFGGGTKVEIK

SEQ ID NO: 21 - DNA, 333 bp, synthetic construct
  misc_feature 1..333: note = source = /note="Description of Artificial Sequence: Synthetic polynucleotide"
  source 1..333: mol_type = other DNA
gatatcgtcctgactcagtcacccgatagcctggccgtcagcctgggcgagcgggctactattaactgtagagctagtgaatcagtcgagtactacggcactagcctgatgcagtggtatcagcagaagcccggtcaaccccctaagctgctgatctacgccgcctctaacgtggaatcaggcgtgcccgataggtttagcggtagcggtagtggcaccgacttcaccctgactattagtagcctgcaggccgaggacgtggccgtctactactgtcagcagtctaggaaggaccctagcaccttcggcggaggcactaaggtcgagattaag

SEQ ID NO: 22 - protein, 218 aa, synthetic construct
  REGION 1..218: note = source = /note="Description of Artificial Sequence: Synthetic polypeptide"
DIVLTQSPDSLAVSLGERATINCRASESVEYYGTSLMQWYQQKPGQPPKLLIYAASNVESGVPDRFSGSGSGTDFTLTISSLQAEDVAVYYCQQSRKDPSTFGGGTKVEIKRTVAAPSVFIFPPSDEQLKSGTASVVCLLNNFYPREAKVQWKVDNALQSGNSQESVTEQDSKDSTYSLSSTLTLSKADYEKHKVYACEVTHQGLSSPVTKSFNRGEC

SEQ ID NO: 23 - DNA, 654 bp, synthetic construct
  misc_feature 1..654: note = source = /note="Description of Artificial Sequence: Synthetic polynucleotide"
  source 1..654: mol_type = other DNA
gatatcgtcctgactcagtcacccgatagcctggccgtcagcctgggcgagcgggctactattaactgtagagctagtgaatcagtcgagtactacggcactagcctgatgcagtggtatcagcagaagcccggtcaaccccctaagctgctgatctacgccgcctctaacgtggaatcaggcgtgcccgataggtttagcggtagcggtagtggcaccgacttcaccctgactattagtagcctgcaggccgaggacgtggccgtctactactgtcagcagtctaggaaggaccctagcaccttcggcggaggcactaaggtcgagattaagcgtacggtggccgctcccagcgtgttcatcttcccccccagcgacgagcagctgaagagcggcaccgccagcgtggtgtgcctgctgaacaacttctacccccgggaggccaaggtgcagtggaaggtggacaacgccctgcagagcggcaacagccaggagagcgtcaccgagcaggacagcaaggactccacctacagcctgagcagcaccctgaccctgagcaaggccgactacgagaagcataaggtgtacgcctgcgaggtgacccaccagggcctgtccagccccgtgaccaagagcttcaacaggggcgagtgc

SEQ ID NO: 24 - protein, 17 aa, synthetic construct
  REGION 1..17: note = source = /note="Description of Artificial Sequence: Synthetic peptide"
DIYPGSGDTSYNQKFKG

SEQ ID NO: 25 - protein, 6 aa, synthetic construct
  REGION 1..6: note = source = /note="Description of Artificial Sequence: Synthetic peptide"
YPGSGD

SEQ ID NO: 26 - protein, 118 aa, synthetic construct
  REGION 1..118: note = source = /note="Description of Artificial Sequence: Synthetic polypeptide"
QVQLVQSGAEVKKPGASVKVSCKASGYTFTSYNMHWVRQAPGQGLEWIGDIYPGSGDTSYNQKFKGRATMTADKSTSTVYMELSSLRSEDTAVYYCARVGGAFPMDYWGQGTLVTVSS

SEQ ID NO: 27 - DNA, 354 bp, synthetic construct
  misc_feature 1..354: note = source = /note="Description of Artificial Sequence: Synthetic polynucleotide"
  source 1..354: mol_type = other DNA
caggtgcagctggtgcagtcaggcgccgaagtgaagaaacccggcgctagtgtgaaagttagctgtaaagctagtggctacaccttcactagctataatatgcactgggttcgccaggccccaggtcaaggcctcgagtggatcggcgatatctaccccggtagcggcgacactagttataatcagaagtttaagggtagagctactatgaccgccgataagtctactagcaccgtctatatggaactgagttccctgaggtctgaagataccgccgtctactactgcgctagagtgggcggagccttccctatggactactggggtcaaggcaccctggtcaccgtgtctagc

SEQ ID NO: 28 - protein, 444 aa, synthetic construct
  REGION 1..444: note = source = /note="Description of Artificial Sequence: Synthetic polypeptide"
QVQLVQSGAEVKKPGASVKVSCKASGYTFTSYNMHWVRQAPGQGLEWIGDIYPGSGDTSYNQKFKGRATMTADKSTSTVYMELSSLRSEDTAVYYCARVGGAFPMDYWGQGTLVTVSSASTKGPSVFPLAPCSRSTSESTAALGCLVKDYFPEPVTVSWNSGALTSGVHTFPAVLQSSGLYSLSSVVTVPSSSLGTKTYTCNVDHKPSNTKVDKRVESKYGPPCPPCPAPEFLGGPSVFLFPPKPKDTLMISRTPEVTCVVVDVSQEDPEVQFNWYVDGVEVHNAKTKPREEQFNSTYRVVSVLTVLHQDWLNGKEYKCKVSNKGLPSSIEKTISKAKGQPREPQVYTLPPSQEEMTKNQVSLTCLVKGFYPSDIAVEWESNGQPENNYKTTPPVLDSDGSFFLYSRLTVDKSRWQEGNVFSCSVMHEALHNHYTQKSLSLSLG

SEQ ID NO: 29 - DNA, 1332 bp, synthetic construct
  misc_feature 1..1332: note = source = /note="Description of Artificial Sequence: Synthetic polynucleotide"
  source 1..1332: mol_type = other DNA
caggtgcagctggtgcagtcaggcgccgaagtgaagaaacccggcgctagtgtgaaagttagctgtaaagctagtggctacaccttcactagctataatatgcactgggttcgccaggccccaggtcaaggcctcgagtggatcggcgatatctaccccggtagcggcgacactagttataatcagaagtttaagggtagagctactatgaccgccgataagtctactagcaccgtctatatggaactgagttccctgaggtctgaagataccgccgtctactactgcgctagagtgggcggagccttccctatggactactggggtcaaggcaccctggtcaccgtgtctagcgctagcactaagggcccgtccgtgttccccctggcaccttgtagccggagcactagcgaatccaccgctgccctcggctgcctggtcaaggattacttcccggagcccgtgaccgtgtcctggaacagcggagccctgacctccggagtgcacaccttccccgctgtgctgcagagctccgggctgtactcgctgtcgtcggtggtcacggtgccttcatctagcctgggtaccaagacctacacttgcaacgtggaccacaagccttccaacactaaggtggacaagcgcgtcgaatcgaagtacggcccaccgtgcccgccttgtcccgcgccggagttcctcggcggtccctcggtctttctgttcccaccgaagcccaaggacactttgatgatttcccgcacccctgaagtgacatgcgtggtcgtggacgtgtcacaggaagatccggaggtgcagttcaattggtacgtggatggcgtcgaggtgcacaacgccaaaaccaagccgagggaggagcagttcaactccacttaccgcgtcgtgtccgtgctgacggtgctgcatcaggactggctgaacgggaaggagtacaagtgcaaagtgtccaacaagggacttcctagctcaatcgaaaagaccatctcgaaagccaagggacagccccgggaaccccaagtgtataccctgccaccgagccaggaagaaatgactaagaaccaagtctcattgacttgccttgtgaagggcttctacccatcggatatcgccgtggaatgggagtccaacggccagccggaaaacaactacaagaccacccctccggtgctggactcagacggatccttcttcctctactcgcggctgaccgtggataagagcagatggcaggagggaaatgtgttcagctgttctgtgatgcatgaagccctgcacaaccactacactcagaagtccctgtccctctccctggga

SEQ ID NO: 30 - protein, 17 aa, synthetic construct
  REGION 1..17: note = source = /note="Description of Artificial Sequence: Synthetic peptide"
DIYPGQGDTSYNQKFKG

SEQ ID NO: 31 - protein, 6 aa, synthetic construct
  REGION 1..6: note = source = /note="Description of Artificial Sequence: Synthetic peptide"
YPGQGD

SEQ ID NO: 32 - protein, 118 aa, synthetic construct
  REGION 1..118: note = source = /note="Description of Artificial Sequence: Synthetic polypeptide"
QVQLVQSGAEVKKPGASVKVSCKASGYTFTSYNMHWVRQAPGQGLEWIGDIYPGQGDTSYNQKFKGRATMTADKSTSTVYMELSSLRSEDTAVYYCARVGGAFPMDYWGQGTLVTVSS

SEQ ID NO: 33 - DNA, 354 bp, synthetic construct
  misc_feature 1..354: note = source = /note="Description of Artificial Sequence: Synthetic polynucleotide"
  source 1..354: mol_type = other DNA
caggtgcagctggtgcagtcaggcgccgaagtgaagaaacccggcgctagtgtgaaagttagctgtaaagctagtggctatactttcacttcttataatatgcactgggtccgccaggccccaggtcaaggcctcgagtggatcggcgatatctaccccggtcaaggcgacacttcctataatcagaagtttaagggtagagctactatgaccgccgataagtctacttctaccgtctatatggaactgagttccctgaggtctgaggacaccgccgtctactactgcgctagagtgggcggagccttcccaatggactactggggtcaaggcaccctggtcaccgtgtctagc

SEQ ID NO: 34 - protein, 444 aa, synthetic construct
  REGION 1..444: note = source = /note="Description of Artificial Sequence: Synthetic polypeptide"
QVQLVQSGAEVKKPGASVKVSCKASGYTFTSYNMHWVRQAPGQGLEWIGDIYPGQGDTSYNQKFKGRATMTADKSTSTVYMELSSLRSEDTAVYYCARVGGAFPMDYWGQGTLVTVSSASTKGPSVFPLAPCSRSTSESTAALGCLVKDYFPEPVTVSWNSGALTSGVHTFPAVLQSSGLYSLSSVVTVPSSSLGTKTYTCNVDHKPSNTKVDKRVESKYGPPCPPCPAPEFLGGPSVFLFPPKPKDTLMISRTPEVTCVVVDVSQEDPEVQFNWYVDGVEVHNAKTKPREEQFNSTYRVVSVLTVLHQDWLNGKEYKCKVSNKGLPSSIEKTISKAKGQPREPQVYTLPPSQEEMTKNQVSLTCLVKGFYPSDIAVEWESNGQPENNYKTTPPVLDSDGSFFLYSRLTVDKSRWQEGNVFSCSVMHEALHNHYTQKSLSLSLG

SEQ ID NO: 35 - DNA, 1332 bp, synthetic construct
  misc_feature 1..1332: note = source = /note="Description of Artificial Sequence: Synthetic polynucleotide"
  source 1..1332: mol_type = other DNA
caggtgcagctggtgcagtcaggcgccgaagtgaagaaacccggcgctagtgtgaaagttagctgtaaagctagtggctatactttcacttcttataatatgcactgggtccgccaggccccaggtcaaggcctcgagtggatcggcgatatctaccccggtcaaggcgacacttcctataatcagaagtttaagggtagagctactatgaccgccgataagtctacttctaccgtctatatggaactgagttccctgaggtctgaggacaccgccgtctactactgcgctagagtgggcggagccttcccaatggactactggggtcaaggcaccctggtcaccgtgtctagcgctagcactaagggcccgtccgtgttccccctggcaccttgtagccggagcactagcgaatccaccgctgccctcggctgcctggtcaaggattacttcccggagcccgtgaccgtgtcctggaacagcggagccctgacctccggagtgcacaccttccccgctgtgctgcagagctccgggctgtactcgctgtcgtcggtggtcacggtgccttcatctagcctgggtaccaagacctacacttgcaacgtggaccacaagccttccaacactaaggtggacaagcgcgtcgaatcgaagtacggcccaccgtgcccgccttgtcccgcgccggagttcctcggcggtccctcggtctttctgttcccaccgaagcccaaggacactttgatgatttcccgcacccctgaagtgacatgcgtggtcgtggacgtgtcacaggaagatccggaggtgcagttcaattggtacgtggatggcgtcgaggtgcacaacgccaaaaccaagccgagggaggagcagttcaactccacttaccgcgtcgtgtccgtgctgacggtgctgcatcaggactggctgaacgggaaggagtacaagtgcaaagtgtccaacaagggacttcctagctcaatcgaaaagaccatctcgaaagccaagggacagccccgggaaccccaagtgtataccctgccaccgagccaggaagaaatgactaagaaccaagtctcattgacttgccttgtgaagggcttctacccatcggatatcgccgtggaatgggagtccaacggccagccggaaaacaactacaagaccacccctccggtgctggactcagacggatccttcttcctctactcgcggctgaccgtggataagagcagatggcaggagggaaatgtgttcagctgttctgtgatgcatgaagccctgcacaaccactacactcagaagtccctgtccctctccctggga

SEQ ID NO: 36 - protein, 118 aa, synthetic construct
  REGION 1..118: note = source = /note="Description of Artificial Sequence: Synthetic polypeptide"
QVQLVQSGAEVKKPGASVKVSCKASGYTFTSYNMHWIRQAPGQGLEWIGDIYPGNGDTSYNQKFKGRATLTADKSTSTVYMELSSLRSEDTAVYYCARVGGAFPMDYWGQGTLVTVSS

SEQ ID NO: 37 - DNA, 354 bp, synthetic construct
  misc_feature 1..354: note = source = /note="Description of Artificial Sequence: Synthetic polynucleotide"
  source 1..354: mol_type = other DNA
caggtgcagctggtgcagtcaggcgccgaagtgaagaaacccggcgctagtgtgaaagtttcttgtaaagctagtggctacaccttcactagctataatatgcactggattagacaggccccagggcagggcctcgagtggatcggcgatatctaccccgggaacggcgacactagttataatcagaagtttaagggtagagctaccctgaccgccgataagtctactagcaccgtctatatggaactgagttccctgaggtctgaggacaccgccgtctactactgcgctagagtgggcggagccttccctatggactactgggggcagggcaccctggtcaccgtgtctagc

SEQ ID NO: 38 - protein, 444 aa, synthetic construct
  REGION 1..444: note = source = /note="Description of Artificial Sequence: Synthetic polypeptide"
QVQLVQSGAEVKKPGASVKVSCKASGYTFTSYNMHWIRQAPGQGLEWIGDIYPGNGDTSYNQKFKGRATLTADKSTSTVYMELSSLRSEDTAVYYCARVGGAFPMDYWGQGTLVTVSSASTKGPSVFPLAPCSRSTSESTAALGCLVKDYFPEPVTVSWNSGALTSGVHTFPAVLQSSGLYSLSSVVTVPSSSLGTKTYTCNVDHKPSNTKVDKRVESKYGPPCPPCPAPEFLGGPSVFLFPPKPKDTLMISRTPEVTCVVVDVSQEDPEVQFNWYVDGVEVHNAKTKPREEQFNSTYRVVSVLTVLHQDWLNGKEYKCKVSNKGLPSSIEKTISKAKGQPREPQVYTLPPSQEEMTKNQVSLTCLVKGFYPSDIAVEWESNGQPENNYKTTPPVLDSDGSFFLYSRLTVDKSRWQEGNVFSCSVMHEALHNHYTQKSLSLSLG

SEQ ID NO: 39 - DNA, 1332 bp, synthetic construct
  misc_feature 1..1332: note = source = /note="Description of Artificial Sequence: Synthetic polynucleotide"
  source 1..1332: mol_type = other DNA
caggtgcagctggtgcagtcaggcgccgaagtgaagaaacccggcgctagtgtgaaagtttcttgtaaagctagtggctacaccttcactagctataatatgcactggattagacaggccccagggcagggcctcgagtggatcggcgatatctaccccgggaacggcgacactagttataatcagaagtttaagggtagagctaccctgaccgccgataagtctactagcaccgtctatatggaactgagttccctgaggtctgaggacaccgccgtctactactgcgctagagtgggcggagccttccctatggactactgggggcagggcaccctggtcaccgtgtctagcgctagcactaagggcccgtccgtgttccccctggcaccttgtagccggagcactagcgaatccaccgctgccctcggctgcctggtcaaggattacttcccggagcccgtgaccgtgtcctggaacagcggagccctgacctccggagtgcacaccttccccgctgtgctgcagagctccgggctgtactcgctgtcgtcggtggtcacggtgccttcatctagcctgggtaccaagacctacacttgcaacgtggaccacaagccttccaacactaaggtggacaagcgcgtcgaatcgaagtacggcccaccgtgcccgccttgtcccgcgccggagttcctcggcggtccctcggtctttctgttcccaccgaagcccaaggacactttgatgatttcccgcacccctgaagtgacatgcgtggtcgtggacgtgtcacaggaagatccggaggtgcagttcaattggtacgtggatggcgtcgaggtgcacaacgccaaaaccaagccgagggaggagcagttcaactccacttaccgcgtcgtgtccgtgctgacggtgctgcatcaggactggctgaacgggaaggagtacaagtgcaaagtgtccaacaagggacttcctagctcaatcgaaaagaccatctcgaaagccaagggacagccccgggaaccccaagtgtataccctgccaccgagccaggaagaaatgactaagaaccaagtctcattgacttgccttgtgaagggcttctacccatcggatatcgccgtggaatgggagtccaacggccagccggaaaacaactacaagaccacccctccggtgctggactcagacggatccttcttcctctactcgcggctgaccgtggataagagcagatggcaggagggaaatgtgttcagctgttctgtgatgcatgaagccctgcacaaccactacactcagaagtccctgtccctctccctggga

SEQ ID NO: 40 - protein, 111 aa, synthetic construct
  REGION 1..111: note = source = /note="Description of Artificial Sequence: Synthetic polypeptide"
DIVLTQSPDSLAVSLGERATINCRASESVEYYGTSLMQWYQQKPGQPPKLLIYAASNVESGVPDRFSGSGSGTDFTLTISSLQAEDVAVYFCQQSRKDPSTFGGGTKVEIK

SEQ ID NO: 41 - DNA, 333 bp, synthetic construct
  misc_feature 1..333: note = source = /note="Description of Artificial Sequence: Synthetic polynucleotide"
  source 1..333: mol_type = other DNA
gatatcgtcctgactcagtcacccgatagcctggccgtcagcctgggcgagcgggctactattaactgtagagctagtgaatcagtcgagtactacggcactagcctgatgcagtggtatcagcagaagcccggtcaaccccctaagctgctgatctacgccgcctctaacgtggaatcaggcgtgcccgataggtttagcggtagcggtagtggcaccgacttcaccctgactattagtagcctgcaggccgaggacgtggccgtctacttctgtcagcagtctaggaaggaccctagcaccttcggcggaggcactaaggtcgagattaag

SEQ ID NO: 42 - protein, 218 aa, synthetic construct
  REGION 1..218: note = source = /note="Description of Artificial Sequence: Synthetic polypeptide"
DIVLTQSPDSLAVSLGERATINCRASESVEYYGTSLMQWYQQKPGQPPKLLIYAASNVESGVPDRFSGSGSGTDFTLTISSLQAEDVAVYFCQQSRKDPSTFGGGTKVEIKRTVAAPSVFIFPPSDEQLKSGTASVVCLLNNFYPREAKVQWKVDNALQSGNSQESVTEQDSKDSTYSLSSTLTLSKADYEKHKVYACEVTHQGLSSPVTKSFNRGEC

SEQ ID NO: 43 - DNA, 654 bp, synthetic construct
  misc_feature 1..654: note = source = /note="Description of Artificial Sequence: Synthetic polynucleotide"
  source 1..654: mol_type = other DNA
gatatcgtcctgactcagtcacccgatagcctggccgtcagcctgggcgagcgggctactattaactgtagagctagtgaatcagtcgagtactacggcactagcctgatgcagtggtatcagcagaagcccggtcaaccccctaagctgctgatctacgccgcctctaacgtggaatcaggcgtgcccgataggtttagcggtagcggtagtggcaccgacttcaccctgactattagtagcctgcaggccgaggacgtggccgtctacttctgtcagcagtctaggaaggaccctagcaccttcggcggaggcactaaggtcgagattaagcgtacggtggccgctcccagcgtgttcatcttcccccccagcgacgagcagctgaagagcggcaccgccagcgtggtgtgcctgctgaacaacttctacccccgggaggccaaggtgcagtggaaggtggacaacgccctgcagagcggcaacagccaggagagcgtcaccgagcaggacagcaaggactccacctacagcctgagcagcaccctgaccctgagcaaggccgactacgagaagcataaggtgtacgcctgcgaggtgacccaccagggcctgtccagccccgtgaccaagagcttcaacaggggcgagtgc

SEQ ID NO: 44 - protein, 118 aa, synthetic construct
  REGION 1..118: note = source = /note="Description of Artificial Sequence: Synthetic polypeptide"
QVQLVQSGAEVKKPGASVKVSCKASGYTFTSYNMHWIRQAPGQGLEWIGDIYPGSGDTSYNQKFKGRATLTADKSTSTVYMELSSLRSEDTAVYYCARVGGAFPMDYWGQGTLVTVSS

SEQ ID NO: 45 - DNA, 354 bp, synthetic construct
  misc_feature 1..354: note = source = /note="Description of Artificial Sequence: Synthetic polynucleotide"
  source 1..354: mol_type = other DNA
caggtgcagctggtgcagtcaggcgccgaagtgaagaaacccggcgcaagcgttaaagtctcatgtaaagctagtggctacaccttcactagctataatatgcactggattagacaggccccagggcaaggcctggagtggatcggcgatatctaccccggtagcggcgacactagttataatcagaagtttaagggtagagctaccctgaccgccgataagtctactagcaccgtctatatggaactgagttccctgaggagtgaagacaccgccgtctactactgcgctagagtgggcggagccttccctatggactactggggtcaaggcaccctggtcaccgtgtcaagc

SEQ ID NO: 46 - protein, 444 aa, synthetic construct
  REGION 1..444: note = source = /note="Description of Artificial Sequence: Synthetic polypeptide"
QVQLVQSGAEVKKPGASVKVSCKASGYTFTSYNMHWIRQAPGQGLEWIGDIYPGSGDTSYNQKFKGRATLTADKSTSTVYMELSSLRSEDTAVYYCARVGGAFPMDYWGQGTLVTVSSASTKGPSVFPLAPCSRSTSESTAALGCLVKDYFPEPVTVSWNSGALTSGVHTFPAVLQSSGLYSLSSVVTVPSSSLGTKTYTCNVDHKPSNTKVDKRVESKYGPPCPPCPAPEFLGGPSVFLFPPKPKDTLMISRTPEVTCVVVDVSQEDPEVQFNWYVDGVEVHNAKTKPREEQFNSTYRVVSVLTVLHQDWLNGKEYKCKVSNKGLPSSIEKTISKAKGQPREPQVYTLPPSQEEMTKNQVSLTCLVKGFYPSDIAVEWESNGQPENNYKTTPPVLDSDGSFFLYSRLTVDKSRWQEGNVFSCSVMHEALHNHYTQKSLSLSLG

SEQ ID NO: 47 - DNA, 1332 bp, synthetic construct
  misc_feature 1..1332: note = source = /note="Description of Artificial Sequence: Synthetic polynucleotide"
  source 1..1332: mol_type = other DNA
caggtgcagctggtgcagtcaggcgccgaagtgaagaaacccggcgcaagcgttaaagtctcatgtaaagctagtggctacaccttcactagctataatatgcactggattagacaggccccagggcaaggcctggagtggatcggcgatatctaccccggtagcggcgacactagttataatcagaagtttaagggtagagctaccctgaccgccgataagtctactagcaccgtctatatggaactgagttccctgaggagtgaagacaccgccgtctactactgcgctagagtgggcggagccttccctatggactactggggtcaaggcaccctggtcaccgtgtcaagcgctagcactaagggcccgtccgtgttccccctggcaccttgtagccggagcactagcgaatccaccgctgccctcggctgcctggtcaaggattacttcccggagcccgtgaccgtgtcctggaacagcggagccctgacctccggagtgcacaccttccccgctgtgctgcagagctccgggctgtactcgctgtcgtcggtggtcacggtgccttcatctagcctgggtaccaagacctacacttgcaacgtggaccacaagccttccaacactaaggtggacaagcgcgtcgaatcgaagtacggcccaccgtgcccgccttgtcccgcgccggagttcctcggcggtccctcggtctttctgttcccaccgaagcccaaggacactttgatgatttcccgcacccctgaagtgacatgcgtggtcgtggacgtgtcacaggaagatccggaggtgcagttcaattggtacgtggatggcgtcgaggtgcacaacgccaaaaccaagccgagggaggagcagttcaactccacttaccgcgtcgtgtccgtgctgacggtgctgcatcaggactggctgaacgggaaggagtacaagtgcaaagtgtccaacaagggacttcctagctcaatcgaaaagaccatctcgaaagccaagggacagccccgggaaccccaagtgtataccctgccaccgagccaggaagaaatgactaagaaccaagtctcattgacttgccttgtgaagggcttctacccatcggatatcgccgtggaatgggagtccaacggccagccggaaaacaactacaagaccacccctccggtgctggactcagacggatccttcttcctctactcgcggctgaccgtggataagagcagatggcaggagggaaatgtgttcagctgttctgtgatgcatgaagccctgcacaaccactacactcagaagtccctgtccctctccctggga

SEQ ID NO: 48 - protein, 118 aa, synthetic construct
  REGION 1..118: note = source = /note="Description of Artificial Sequence: Synthetic polypeptide"
QVQLVQSGAEVKKPGASVKVSCKASGYTFTSYNMHWIRQAPGQGLEWIGDIYPGQGDTSYNQKFKGRATLTADKSTSTVYMELSSLRSEDTAVYYCARVGGAFPMDYWGQGTLVTVSS

SEQ ID NO: 49 - DNA, 354 bp, synthetic construct
  misc_feature 1..354: note = source = /note="Description of Artificial Sequence: Synthetic polynucleotide"
  source 1..354: mol_type = other DNA
caggtgcagctggtgcagtcaggcgccgaagtgaagaaacccggcgctagtgtgaaagtctcttgtaaagctagtggctacaccttcactagctataatatgcactggattagacaggccccaggtcaaggcctcgagtggatcggcgatatctaccccggtcaaggcgacactagttataatcagaagtttaagggtagagctaccctgaccgccgataagtctactagcaccgtctatatggaactgagttccctgaggtctgaggacaccgccgtctactactgcgctagagtgggcggagccttccctatggactactggggtcaaggcaccctggtcaccgtgtctagc

SEQ ID NO: 50 - protein, 444 aa, synthetic construct
  REGION 1..444: note = source = /note="Description of Artificial Sequence: Synthetic polypeptide"
QVQLVQSGAEVKKPGASVKVSCKASGYTFTSYNMHWIRQAPGQGLEWIGDIYPGQGDTSYNQKFKGRATLTADKSTSTVYMELSSLRSEDTAVYYCARVGGAFPMDYWGQGTLVTVSSASTKGPSVFPLAPCSRSTSESTAALGCLVKDYFPEPVTVSWNSGALTSGVHTFPAVLQSSGLYSLSSVVTVPSSSLGTKTYTCNVDHKPSNTKVDKRVESKYGPPCPPCPAPEFLGGPSVFLFPPKPKDTLMISRTPEVTCVVVDVSQEDPEVQFNWYVDGVEVHNAKTKPREEQFNSTYRVVSVLTVLHQDWLNGKEYKCKVSNKGLPSSIEKTISKAKGQPREPQVYTLPPSQEEMTKNQVSLTCLVKGFYPSDIAVEWESNGQPENNYKTTPPVLDSDGSFFLYSRLTVDKSRWQEGNVFSCSVMHEALHNHYTQKSLSLSLG

SEQ ID NO: 51 - DNA, 1332 bp, synthetic construct
  misc_feature 1..1332: note = source = /note="Description of Artificial Sequence: Synthetic polynucleotide"
  source 1..1332: mol_type = other DNA
caggtgcagctggtgcagtcaggcgccgaagtgaagaaacccggcgctagtgtgaaagtctcttgtaaagctagtggctacaccttcactagctataatatgcactggattagacaggccccaggtcaaggcctcgagtggatcggcgatatctaccccggtcaaggcgacactagttataatcagaagtttaagggtagagctaccctgaccgccgataagtctactagcaccgtctatatggaactgagttccctgaggtctgaggacaccgccgtctactactgcgctagagtgggcggagccttccctatggactactggggtcaaggcaccctggtcaccgtgtctagcgctagcactaagggcccgtccgtgttccccctggcaccttgtagccggagcactagcgaatccaccgctgccctcggctgcctggtcaaggattacttcccggagcccgtgaccgtgtcctggaacagcggagccctgacctccggagtgcacaccttccccgctgtgctgcagagctccgggctgtactcgctgtcgtcggtggtcacggtgccttcatctagcctgggtaccaagacctacacttgcaacgtggaccacaagccttccaacactaaggtggacaagcgcgtcgaatcgaagtacggcccaccgtgcccgccttgtcccgcgccggagttcctcggcggtccctcggtctttctgttcccaccgaagcccaaggacactttgatgatttcccgcacccctgaagtgacatgcgtggtcgtggacgtgtcacaggaagatccggaggtgcagttcaattggtacgtggatggcgtcgaggtgcacaacgccaaaaccaagccgagggaggagcagttcaactccacttaccgcgtcgtgtccgtgctgacggtgctgcatcaggactggctgaacgggaaggagtacaagtgcaaagtgtccaacaagggacttcctagctcaatcgaaaagaccatctcgaaagccaagggacagccccgggaaccccaagtgtataccctgccaccgagccaggaagaaatgactaagaaccaagtctcattgacttgccttgtgaagggcttctacccatcggatatcgccgtggaatgggagtccaacggccagccggaaaacaactacaagaccacccctccggtgctggactcagacggatccttcttcctctactcgcggctgaccgtggataagagcagatggcaggagggaaatgtgttcagctgttctgtgatgcatgaagccctgcacaaccactacactcagaagtccctgtccctctccctggga

SEQ ID NO: 52 - protein, 118 aa, synthetic construct
  REGION 1..118: note = source = /note="Description of Artificial Sequence: Synthetic polypeptide"
QVQLVQSGAEVKKPGSSVKVSCKASGYTFTSYNMHWVRQAPGQGLEWMGDIYPGNGDTSYNQKFKGRVTITADKSTSTVYMELSSLRSEDTAVYYCARVGGAFPMDYWGQGTTVTVSS

SEQ ID NO: 53 - DNA, 354 bp, synthetic construct
  misc_feature 1..354: note = source = /note="Description of Artificial Sequence: Synthetic polynucleotide"
  source 1..354: mol_type = other DNA
caggtgcagctggtgcagtcaggcgccgaagtgaagaaacccggctctagcgtgaaagtttcttgtaaagctagtggctacaccttcactagctataatatgcactgggttcgccaggccccagggcaaggcctcgagtggatgggcgatatctaccccgggaacggcgacactagttataatcagaagtttaagggtagagtcactatcaccgccgataagtctactagcaccgtctatatggaactgagttccctgaggtctgaggacaccgccgtctactactgcgctagagtgggcggagccttccctatggactactggggtcaaggcactaccgtgaccgtgtctagc

SEQ ID NO: 54 - protein, 444 aa, synthetic construct
  REGION 1..444: note = source = /note="Description of Artificial Sequence: Synthetic polypeptide"
QVQLVQSGAEVKKPGSSVKVSCKASGYTFTSYNMHWVRQAPGQGLEWMGDIYPGNGDTSYNQKFKGRVTITADKSTSTVYMELSSLRSEDTAVYYCARVGGAFPMDYWGQGTTVTVSSASTKGPSVFPLAPCSRSTSESTAALGCLVKDYFPEPVTVSWNSGALTSGVHTFPAVLQSSGLYSLSSVVTVPSSSLGTKTYTCNVDHKPSNTKVDKRVESKYGPPCPPCPAPEFLGGPSVFLFPPKPKDTLMISRTPEVTCVVVDVSQEDPEVQFNWYVDGVEVHNAKTKPREEQFNSTYRVVSVLTVLHQDWLNGKEYKCKVSNKGLPSSIEKTISKAKGQPREPQVYTLPPSQEEMTKNQVSLTCLVKGFYPSDIAVEWESNGQPENNYKTTPPVLDSDGSFFLYSRLTVDKSRWQEGNVFSCSVMHEALHNHYTQKSLSLSLG

SEQ ID NO: 55 - DNA, 1332 bp, synthetic construct
  misc_feature 1..1332: note = source = /note="Description of Artificial Sequence: Synthetic polynucleotide"
  source 1..1332: mol_type = other DNA
caggtgcagctggtgcagtcaggcgccgaagtgaagaaacccggctctagcgtgaaagtttcttgtaaagctagtggctacaccttcactagctataatatgcactgggttcgccaggccccagggcaaggcctcgagtggatgggcgatatctaccccgggaacggcgacactagttataatcagaagtttaagggtagagtcactatcaccgccgataagtctactagcaccgtctatatggaactgagttccctgaggtctgaggacaccgccgtctactactgcgctagagtgggcggagccttccctatggactactggggtcaaggcactaccgtgaccgtgtctagcgctagcactaagggcccgtccgtgttccccctggcaccttgtagccggagcactagcgaatccaccgctgccctcggctgcctggtcaaggattacttcccggagcccgtgaccgtgtcctggaacagcggagccctgacctccggagtgcacaccttccccgctgtgctgcagagctccgggctgtactcgctgtcgtcggtggtcacggtgccttcatctagcctgggtaccaagacctacacttgcaacgtggaccacaagccttccaacactaaggtggacaagcgcgtcgaatcgaagtacggcccaccgtgcccgccttgtcccgcgccggagttcctcggcggtccctcggtctttctgttcccaccgaagcccaaggacactttgatgatttcccgcacccctgaagtgacatgcgtggtcgtggacgtgtcacaggaagatccggaggtgcagttcaattggtacgtggatggcgtcgaggtgcacaacgccaaaaccaagccgagggaggagcagttcaactccacttaccgcgtcgtgtccgtgctgacggtgctgcatcaggactggctgaacgggaaggagtacaagtgcaaagtgtccaacaagggacttcctagctcaatcgaaaagaccatctcgaaagccaagggacagccccgggaaccccaagtgtataccctgccaccgagccaggaagaaatgactaagaaccaagtctcattgacttgccttgtgaagggcttctacccatcggatatcgccgtggaatgggagtccaacggccagccggaaaacaactacaagaccacccctccggtgctggactcagacggatccttcttcctctactcgcggctgaccgtggataagagcagatggcaggagggaaatgtgttcagctgttctgtgatgcatgaagccctgcacaaccactacactcagaagtccctgtccctctccctggga

SEQ ID NO: 56 - protein, 111 aa, synthetic construct
  REGION 1..111: note = source = /note="Description of Artificial Sequence: Synthetic polypeptide"
EIVLTQSPATLSLSPGERATLSCRASESVEYYGTSLMQWYQQKPGQAPRLLIYAASNVESGIPARFSGSGSGTDFTLTISSLEPEDIAVYFCQQSRKDPSTFGGGTKVEIK

SEQ ID NO: 57 - DNA, 333 bp, synthetic construct
  misc_feature 1..333: note = source = /note="Description of Artificial Sequence: Synthetic polynucleotide"
  source 1..333: mol_type = other DNA
gagatcgtcctgactcagtcacccgctaccctgagcctgagccctggcgagagagctacactgagctgtagagctagtgaatcagtcgagtactacggcactagcctgatgcagtggtatcagcagaagcccggtcaagcccctagactgctgatctacgccgcctctaacgtggaatcagggatccccgctaggtttagcggtagcggtagtggcaccgacttcaccctgactatctctagcctggaacccgaggatatcgccgtctacttctgtcagcagtctaggaaggaccctagcaccttcggcggaggcactaaggtcgagattaag

SEQ ID NO: 58 - protein, 218 aa, synthetic construct
  REGION 1..218: note = source = /note="Description of Artificial Sequence: Synthetic polypeptide"
EIVLTQSPATLSLSPGERATLSCRASESVEYYGTSLMQWYQQKPGQAPRLLIYAASNVESGIPARFSGSGSGTDFTLTISSLEPEDIAVYFCQQSRKDPSTFGGGTKVEIKRTVAAPSVFIFPPSDEQLKSGTASVVCLLNNFYPREAKVQWKVDNALQSGNSQESVTEQDSKDSTYSLSSTLTLSKADYEKHKVYACEVTHQGLSSPVTKSFNRGEC

SEQ ID NO: 59 - DNA, 654 bp, synthetic construct
  misc_feature 1..654: note = source = /note="Description of Artificial Sequence: Synthetic polynucleotide"
  source 1..654: mol_type = other DNA
gagatcgtcctgactcagtcacccgctaccctgagcctgagccctggcgagagagctacactgagctgtagagctagtgaatcagtcgagtactacggcactagcctgatgcagtggtatcagcagaagcccggtcaagcccctagactgctgatctacgccgcctctaacgtggaatcagggatccccgctaggtttagcggtagcggtagtggcaccgacttcaccctgactatctctagcctggaacccgaggatatcgccgtctacttctgtcagcagtctaggaaggaccctagcaccttcggcggaggcactaaggtcgagattaagcgtacggtggccgctcccagcgtgttcatcttcccccccagcgacgagcagctgaagagcggcaccgccagcgtggtgtgcctgctgaacaacttctacccccgggaggccaaggtgcagtggaaggtggacaacgccctgcagagcggcaacagccaggagagcgtcaccgagcaggacagcaaggactccacctacagcctgagcagcaccctgaccctgagcaaggccgactacgagaagcataaggtgtacgcctgcgaggtgacccaccagggcctgtccagccccgtgaccaagagcttcaacaggggcgagtgc

SEQ ID NO: 60 - protein, 118 aa, synthetic construct
  REGION 1..118: note = source = /note="Description of Artificial Sequence: Synthetic polypeptide"
EVQLVQSGAEVKKPGESLKISCKGSGYTFTSYNMHWVRQMPGKGLEWMGDIYPGNGDTSYNQKFKGQVTISADKSISTVYLQWSSLKASDTAMYYCARVGGAFPMDYWGQGTTVTVSS

SEQ ID NO: 61 - DNA, 354 bp, synthetic construct
  misc_feature 1..354: note = source = /note="Description of Artificial Sequence: Synthetic polynucleotide"
  source 1..354: mol_type = other DNA
gaagtgcagctggtgcagtcaggcgccgaagtgaagaagcccggcgagtcactgaagattagctgtaaaggttcaggctacaccttcactagctataatatgcactgggtccgccagatgcccgggaaaggcctcgagtggatgggcgatatctaccccgggaacggcgacactagttataatcagaagtttaaggggcaagtcacaattagcgccgataagtctattagcaccgtctacctgcagtggtctagcctgaaggctagtgacaccgctatgtactactgcgctagagtgggcggagccttccctatggactactggggtcaaggcactaccgtgaccgtgtctagc

SEQ ID NO: 62 - protein, 444 aa, synthetic construct
  REGION 1..444: note = source = /note="Description of Artificial Sequence: Synthetic polypeptide"
EVQLVQSGAEVKKPGESLKISCKGSGYTFTSYNMHWVRQMPGKGLEWMGDIYPGNGDTSYNQKFKGQVTISADKSISTVYLQWSSLKASDTAMYYCARVGGAFPMDYWGQGTTVTVSSASTKGPSVFPLAPCSRSTSESTAALGCLVKDYFPEPVTVSWNSGALTSGVHTFPAVLQSSGLYSLSSVVTVPSSSLGTKTYTCNVDHKPSNTKVDKRVESKYGPPCPPCPAPEFLGGPSVFLFPPKPKDTLMISRTPEVTCVVVDVSQEDPEVQFNWYVDGVEVHNAKTKPREEQFNSTYRVVSVLTVLHQDWLNGKEYKCKVSNKGLPSSIEKTISKAKGQPREPQVYTLPPSQEEMTKNQVSLTCLVKGFYPSDIAVEWESNGQPENNYKTTPPVLDSDGSFFLYSRLTVDKSRWQEGNVFSCSVMHEALHNHYTQKSLSLSLG

SEQ ID NO: 63 - DNA, 1332 bp, synthetic construct
  misc_feature 1..1332: note = source = /note="Description of Artificial Sequence: Synthetic polynucleotide"
  source 1..1332: mol_type = other DNA
gaagtgcagctggtgcagtcaggcgccgaagtgaagaagcccggcgagtcactgaagattagctgtaaaggttcaggctacaccttcactagctataatatgcactgggtccgccagatgcccgggaaaggcctcgagtggatgggcgatatctaccccgggaacggcgacactagttataatcagaagtttaaggggcaagtcacaattagcgccgataagtctattagcaccgtctacctgcagtggtctagcctgaaggctagtgacaccgctatgtactactgcgctagagtgggcggagccttccctatggactactggggtcaaggcactaccgtgaccgtgtctagcgctagcactaagggcccgtccgtgttccccctggcaccttgtagccggagcactagcgaatccaccgctgccctcggctgcctggtcaaggattacttcccggagcccgtgaccgtgtcctggaacagcggagccctgacctccggagtgcacaccttccccgctgtgctgcagagctccgggctgtactcgctgtcgtcggtggtcacggtgccttcatctagcctgggtaccaagacctacacttgcaacgtggaccacaagccttccaacactaaggtggacaagcgcgtcgaatcgaagtacggcccaccgtgcccgccttgtcccgcgccggagttcctcggcggtccctcggtctttctgttcccaccgaagcccaaggacactttgatgatttcccgcacccctgaagtgacatgcgtggtcgtggacgtgtcacaggaagatccggaggtgcagttcaattggtacgtggatggcgtcgaggtgcacaacgccaaaaccaagccgagggaggagcagttcaactccacttaccgcgtcgtgtccgtgctgacggtgctgcatcaggactggctgaacgggaaggagtacaagtgcaaagtgtccaacaagggacttcctagctcaatcgaaaagaccatctcgaaagccaagggacagccccgggaaccccaagtgtataccctgccaccgagccaggaagaaatgactaagaaccaagtctcattgacttgccttgtgaagggcttctacccatcggatatcgccgtggaatgggagtccaacggccagccggaaaacaactacaagaccacccctccggtgctggactcagacggatccttcttcctctactcgcggctgaccgtggataagagcagatggcaggagggaaatgtgttcagctgttctgtgatgcatgaagccctgcacaaccactacactcagaagtccctgtccctctccctggga

SEQ ID NO: 64 - protein, 111 aa, synthetic construct
  REGION 1..111: note = source = /note="Description of Artificial Sequence: Synthetic polypeptide"
AIQLTQSPSSLSASVGDRVTITCRASESVEYYGTSLMQWYQQKPGKAPKLLIYAASNVESGVPSRFSGSGSGTDFTLTISSLQPEDFATYFCQQSRKDPSTFGGGTKVEIK

SEQ ID NO: 65 - DNA, 333 bp, synthetic construct
  misc_feature 1..333: note = source = /note="Description of Artificial Sequence: Synthetic polynucleotide"
  source 1..333: mol_type = other DNA
gctattcagctgactcagtcacctagtagcctgagcgctagtgtgggcgatagagtgactatcacctgtagagctagtgaatcagtcgagtactacggcactagcctgatgcagtggtatcagcagaagcccgggaaagcccctaagctgctgatctacgccgcctctaacgtggaatcaggcgtgccctctaggtttagcggtagcggtagtggcaccgacttcaccctgactatctctagcctgcagcccgaggacttcgctacctacttctgtcagcagtctaggaaggaccctagcaccttcggcggaggcactaaggtcgagattaag

SEQ ID NO: 66 - protein, 218 aa, synthetic construct
  REGION 1..218: note = source = /note="Description of Artificial Sequence: Synthetic polypeptide"
AIQLTQSPSSLSASVGDRVTITCRASESVEYYGTSLMQWYQQKPGKAPKLLIYAASNVESGVPSRFSGSGSGTDFTLTISSLQPEDFATYFCQQSRKDPSTFGGGTKVEIKRTVAAPSVFIFPPSDEQLKSGTASVVCLLNNFYPREAKVQWKVDNALQSGNSQESVTEQDSKDSTYSLSSTLTLSKADYEKHKVYACEVTHQGLSSPVTKSFNRGEC

SEQ ID NO: 67 - DNA, 654 bp, synthetic construct
  misc_feature 1..654: note = source = /note="Description of Artificial Sequence: Synthetic polynucleotide"
  source 1..654: mol_type = other DNA
gctattcagctgactcagtcacctagtagcctgagcgctagtgtgggcgatagagtgactatcacctgtagagctagtgaatcagtcgagtactacggcactagcctgatgcagtggtatcagcagaagcccgggaaagcccctaagctgctgatctacgccgcctctaacgtggaatcaggcgtgccctctaggtttagcggtagcggtagtggcaccgacttcaccctgactatctctagcctgcagcccgaggacttcgctacctacttctgtcagcagtctaggaaggaccctagcaccttcggcggaggcactaaggtcgagattaagcgtacggtggccgctcccagcgtgttcatcttcccccccagcgacgagcagctgaagagcggcaccgccagcgtggtgtgcctgctgaacaacttctacccccgggaggccaaggtgcagtggaaggtggacaacgccctgcagagcggcaacagccaggagagcgtcaccgagcaggacagcaaggactccacctacagcctgagcagcaccctgaccctgagcaaggccgactacgagaagcataaggtgtacgcctgcgaggtgacccaccagggcctgtccagccccgtgaccaagagcttcaacaggggcgagtgc

SEQ ID NO: 68 - protein, 118 aa, synthetic construct
  REGION 1..118: note = source = /note="Description of Artificial Sequence: Synthetic polypeptide"
QVQLVQSGAEVKKPGSSVKVSCKASGYTFTSYNMHWVRQAPGQGLEWMGDIYPGSGDTSYNQKFKGRVTITADKSTSTVYMELSSLRSEDTAVYYCARVGGAFPMDYWGQGTTVTVSS

SEQ ID NO: 69 - DNA, 354 bp, synthetic construct
  misc_feature 1..354: note = source = /note="Description of Artificial Sequence: Synthetic polynucleotide"
  source 1..354: mol_type = other DNA
caggtgcaattggttcagtcaggagcagaagttaagaagccaggatcatccgtcaaggtgtcctgcaaagcatctggctacaccttcaccagctacaatatgcactgggtccgacaagcccctgggcagggcttggagtggatgggagacatttaccccggcagtggtgacacttcctataaccagaagttcaagggccgagtcactattaccgctgacaagtccacctccacagtctacatggaactctcttctctgagatccgaggacactgccgtctattactgcgctcgcgtgggcggtgctttcccaatggactattggggacagggcacaaccgtgaccgtcagctca

SEQ ID NO: 70 - protein, 445 aa, synthetic construct
  REGION 1..445: note = source = /note="Description of Artificial Sequence: Synthetic polypeptide"
QVQLVQSGAEVKKPGSSVKVSCKASGYTFTSYNMHWVRQAPGQGLEWMGDIYPGSGDTSYNQKFKGRVTITADKSTSTVYMELSSLRSEDTAVYYCARVGGAFPMDYWGQGTTVTVSSASTKGPSVFPLAPCSRSTSESTAALGCLVKDYFPEPVTVSWNSGALTSGVHTFPAVLQSSGLYSLSSVVTVPSSSLGTKTYTCNVDHKPSNTKVDKRVESKYGPPCPPCPAPEFLGGPSVFLFPPKPKDTLMISRTPEVTCVVVDVSQEDPEVQFNWYVDGVEVHNAKTKPREEQFNSTYRVVSVLTVLHQDWLNGKEYKCKVSNKGLPSSIEKTISKAKGQPREPQVYTLPPSQEEMTKNQVSLTCLVKGFYPSDIAVEWESNGQPENNYKTTPPVLDSDGSFFLYSRLTVDKSRWQEGNVFSCSVMHEALHNHYTQKSLSLSLGK

SEQ ID NO: 71 - DNA, 1335 bp, synthetic construct
  misc_feature 1..1335: note = source = /note="Description of Artificial Sequence: Synthetic polynucleotide"
  source 1..1335: mol_type = other DNA
caggtgcaattggttcagtcaggagcagaagttaagaagccaggatcatccgtcaaggtgtcctgcaaagcatctggctacaccttcaccagctacaatatgcactgggtccgacaagcccctgggcagggcttggagtggatgggagacatttaccccggcagtggtgacacttcctataaccagaagttcaagggccgagtcactattaccgctgacaagtccacctccacagtctacatggaactctcttctctgagatccgaggacactgccgtctattactgcgctcgcgtgggcggtgctttcccaatggactattggggacagggcacaaccgtgaccgtcagctcagcctctacaaagggcccctccgtctttccactcgcgccgtgctctcgctccacctcagagtcaactgccgctctgggttgcctggtcaaggactacttcccagagccggtgacagtgagctggaacagtggggccctgacatccggcgttcataccttccccgcagtcctccagtcctcaggcctgtattccctgagcagcgttgtcacagtgccctccagctctcttggcacgaaaacctacacatgcaacgttgatcataagccgtctaataccaaggtggataaaagagtggagagcaagtacggcccaccctgcccgccttgcccagctccggagttcctgggcggaccatccgttttcttgtttccacccaaacctaaagacactctgatgatttcccgaacccctgaagtgacttgcgttgtggtggacgtctcccaggaggacccagaagtgcaattcaactggtacgtggacggggtggaggtgcacaatgcaaaaaccaaaccaagggaggaacagtttaattcaacatatagggttgtgtctgtgctgacggttctgcatcaggactggctgaacggaaaggaatacaagtgcaaggtgtccaacaaaggactgccaagctctatcgagaaaacaatctctaaggccaagggacaacctagagagccccaagtttacaccctgccaccatcacaggaagagatgaccaaaaatcaggtgagcttgacatgcctggtgaagggcttctaccctagcgatattgcggttgagtgggagtcaaatggccagcctgagaacaactataagactactcctcccgtgctggactccgacgggagctttttcctgtattccaggcttacagtcgataagagcagatggcaagaggggaatgtgttttcctgctccgtgatgcacgaggctctccataaccattatactcagaaaagtctctctctgtcactgggcaaa

SEQ ID NO: 72 - protein, 118 aa, synthetic construct
  REGION 1..118: note = source = /note="Description of Artificial Sequence: Synthetic polypeptide"
QVQLVQSGAEVKKPGSSVKVSCKASGYTFTSYNMHWVRQAPGQGLEWMGDIYPGQGDTSYNQKFKGRVTITADKSTSTVYMELSSLRSEDTAVYYCARVGGAFPMDYWGQGTTVTVSS

SEQ ID NO: 73 - DNA, 354 bp, synthetic construct
  misc_feature 1..354: note = source = /note="Description of Artificial Sequence: Synthetic polynucleotide"
  source 1..354: mol_type = other DNA
caggtgcaattggttcagtcaggagcagaagttaagaagccaggatcatccgtcaaggtgtcctgcaaagcatctggctacaccttcaccagctacaatatgcactgggtccgacaagcccctgggcagggcttggagtggatgggagacatttaccccggccagggtgacacttcctataaccagaagttcaagggccgagtcactattaccgctgacaagtccacctccacagtctacatggaactctcttctctgagatccgaggacactgccgtctattactgcgctcgcgtgggcggtgctttcccaatggactattggggacagggcacaaccgtgaccgtcagctca

SEQ ID NO: 74 - protein, 445 aa, synthetic construct
  REGION 1..445: note = source = /note="Description of Artificial Sequence: Synthetic polypeptide"
QVQLVQSGAEVKKPGSSVKVSCKASGYTFTSYNMHWVRQAPGQGLEWMGDIYPGQGDTSYNQKFKGRVTITADKSTSTVYMELSSLRSEDTAVYYCARVGGAFPMDYWGQGTTVTVSSASTKGPSVFPLAPCSRSTSESTAALGCLVKDYFPEPVTVSWNSGALTSGVHTFPAVLQSSGLYSLSSVVTVPSSSLGTKTYTCNVDHKPSNTKVDKRVESKYGPPCPPCPAPEFLGGPSVFLFPPKPKDTLMISRTPEVTCVVVDVSQEDPEVQFNWYVDGVEVHNAKTKPREEQFNSTYRVVSVLTVLHQDWLNGKEYKCKVSNKGLPSSIEKTISKAKGQPREPQVYTLPPSQEEMTKNQVSLTCLVKGFYPSDIAVEWESNGQPENNYKTTPPVLDSDGSFFLYSRLTVDKSRWQEGNVFSCSVMHEALHNHYTQKSLSLSLGK

SEQ ID NO: 75 - DNA, 1335 bp, synthetic construct
  misc_feature 1..1335: note = source = /note="Description of Artificial Sequence: Synthetic polynucleotide"
  source 1..1335: mol_type = other DNA
caggtgcaattggttcagtcaggagcagaagttaagaagccaggatcatccgtcaaggtgtcctgcaaagcatctggctacaccttcaccagctacaatatgcactgggtccgacaagcccctgggcagggcttggagtggatgggagacatttaccccggccagggtgacacttcctataaccagaagttcaagggccgagtcactattaccgctgacaagtccacctccacagtctacatggaactctcttctctgagatccgaggacactgccgtctattactgcgctcgcgtgggcggtgctttcccaatggactattggggacagggcacaaccgtgaccgtcagctcagcctctacaaagggcccctccgtctttccactcgcgccgtgctctcgctccacctcagagtcaactgccgctctgggttgcctggtcaaggactacttcccagagccggtgacagtgagctggaacagtggggccctgacatccggcgttcataccttccccgcagtcctccagtcctcaggcctgtattccctgagcagcgttgtcacagtgccctccagctctcttggcacgaaaacctacacatgcaacgttgatcataagccgtctaataccaaggtggataaaagagtggagagcaagtacggcccaccctgcccgccttgcccagctccggagttcctgggcggaccatccgttttcttgtttccacccaaacctaaagacactctgatgatttcccgaacccctgaagtgacttgcgttgtggtggacgtctcccaggaggacccagaagtgcaattcaactggtacgtggacggggtggaggtgcacaatgcaaaaaccaaaccaagggaggaacagtttaattcaacatatagggttgtgtctgtgctgacggttctgcatcaggactggctgaacggaaaggaatacaagtgcaaggtgtccaacaaaggactgccaagctctatcgagaaaacaatctctaaggccaagggacaacctagagagccccaagtttacaccctgccaccatcacaggaagagatgaccaaaaatcaggtgagcttgacatgcctggtgaagggcttctaccctagcgatattgcggttgagtgggagtcaaatggccagcctgagaacaactataagactactcctcccgtgctggactccgacgggagctttttcctgtattccaggcttacagtcgataagagcagatggcaagaggggaatgtgttttcctgctccgtgatgcacgaggctctccataaccattatactcagaaaagtctctctctgtcactgggcaaa

SEQ ID NO: 76 - protein, 118 aa, synthetic construct
  REGION 1..118: note = source = /note="Description of Artificial Sequence: Synthetic polypeptide"
EVQLVQSGAEVKKPGESLKISCKGSGYTFTSYNMHWVRQMPGKGLEWMGDIYPGSGDTSYNQKFKGQVTISADKSISTVYLQWSSLKASDTAMYYCARVGGAFPMDYWGQGTTVTVSS

SEQ ID NO: 77 - DNA, 354 bp, synthetic construct
  misc_feature 1..354: note = source = /note="Description of Artificial Sequence: Synthetic polynucleotide"
  source 1..354: mol_type = other DNA
gaagttcaattggtacagtctggcgcagaagtaaagaaaccaggagagagtttgaaaatttcctgcaagggcagtgggtacacattcacgtcctacaatatgcactgggtgagacagatgccaggcaagggcctggagtggatgggagacatatacccaggcagtggagacacaagctataatcagaaattcaaaggacaggtgacgatctccgcagacaaatccatatctacggtctacctccagtggtcctcacttaaagcctccgacaccgccatgtactattgcgctcgggtaggtggcgcgtttccaatggactattggggccaagggaccacagtaaccgtcagctca

SEQ ID NO: 78 - protein, 445 aa, synthetic construct
  REGION 1..445: note = source = /note="Description of Artificial Sequence: Synthetic polypeptide"
EVQLVQSGAEVKKPGESLKISCKGSGYTFTSYNMHWVRQMPGKGLEWMGDIYPGSGDTSYNQKFKGQVTISADKSISTVYLQWSSLKASDTAMYYCARVGGAFPMDYWGQGTTVTVSSASTKGPSVFPLAPCSRSTSESTAALGCLVKDYFPEPVTVSWNSGALTSGVHTFPAVLQSSGLYSLSSVVTVPSSSLGTKTYTCNVDHKPSNTKVDKRVESKYGPPCPPCPAPEFLGGPSVFLFPPKPKDTLMISRTPEVTCVVVDVSQEDPEVQFNWYVDGVEVHNAKTKPREEQFNSTYRVVSVLTVLHQDWLNGKEYKCKVSNKGLPSSIEKTISKAKGQPREPQVYTLPPSQEEMTKNQVSLTCLVKGFYPSDIAVEWESNGQPENNYKTTPPVLDSDGSFFLYSRLTVDKSRWQEGNVFSCSVMHEALHNHYTQKSLSLSLGK

SEQ ID NO: 79 - DNA, 1335 bp, synthetic construct
  misc_feature 1..1335: note = source = /note="Description of Artificial Sequence: Synthetic polynucleotide"
  source 1..1335: mol_type = other DNA
gaagttcaattggtacagtctggcgcagaagtaaagaaaccaggagagagtttgaaaatttcctgcaagggcagtgggtacacattcacgtcctacaatatgcactgggtgagacagatgccaggcaagggcctggagtggatgggagacatatacccaggcagtggagacacaagctataatcagaaattcaaaggacaggtgacgatctccgcagacaaatccatatctacggtctacctccagtggtcctcacttaaagcctccgacaccgccatgtactattgcgctcgggtaggtggcgcgtttccaatggactattggggccaagggaccacagtaaccgtcagctcagcctctacaaagggcccctccgtctttccactcgcgccgtgctctcgctccacctcagagtcaactgccgctctgggttgcctggtcaaggactacttcccagagccggtgacagtgagctggaacagtggggccctgacatccggcgttcataccttccccgcagtcctccagtcctcaggcctgtattccctgagcagcgttgtcacagtgccctccagctctcttggcacgaaaacctacacatgcaacgttgatcataagccgtctaataccaaggtggataaaagagtggagagcaagtacggcccaccctgcccgccttgcccagctccggagttcctgggcggaccatccgttttcttgtttccacccaaacctaaagacactctgatgatttcccgaacccctgaagtgacttgcgttgtggtggacgtctcccaggaggacccagaagtgcaattcaactggtacgtggacggggtggaggtgcacaatgcaaaaaccaaaccaagggaggaacagtttaattcaacatatagggttgtgtctgtgctgacggttctgcatcaggactggctgaacggaaaggaatacaagtgcaaggtgtccaacaaaggactgccaagctctatcgagaaaacaatctctaaggccaagggacaacctagagagccccaagtttacaccctgccaccatcacaggaagagatgaccaaaaatcaggtgagcttgacatgcctggtgaagggcttctaccctagcgatattgcggttgagtgggagtcaaatggccagcctgagaacaactataagactactcctcccgtgctggactccgacgggagctttttcctgtattccaggcttacagtcgataagagcagatggcaagaggggaatgtgttttcctgctccgtgatgcacgaggctctccataaccattatactcagaaaagtctctctctgtcactgggcaaa

SEQ ID NO: 80 - protein, 118 aa, synthetic construct
  REGION 1..118: note = source = /note="Description of Artificial Sequence: Synthetic polypeptide"
EVQLVQSGAEVKKPGESLKISCKGSGYTFTSYNMHWVRQMPGKGLEWMGDIYPGQGDTSYNQKFKGQVTISADKSISTVYLQWSSLKASDTAMYYCARVGGAFPMDYWGQGTTVTVSS

SEQ ID NO: 81 - DNA, 354 bp, synthetic construct
  misc_feature 1..354: note = source = /note="Description of Artificial Sequence: Synthetic polynucleotide"
  source 1..354: mol_type = other DNA
gaagttcaattggtacagtctggcgcagaagtaaagaaaccaggagagagtttgaaaatttcctgcaagggcagtgggtacacattcacgtcctacaatatgcactgggtgagacagatgccaggcaagggcctggagtggatgggagacatatacccaggccagggagacacaagctataatcagaaattcaaaggacaggtgacgatctccgcagacaaatccatatctacggtctacctccagtggtcctcacttaaagcctccgacaccgccatgtactattgcgctcgggtaggtggcgcgtttccaatggactattggggccaagggaccacagtaaccgtcagctca

SEQ ID NO: 82 - protein, 445 aa, synthetic construct
  REGION 1..445: note = source = /note="Description of Artificial Sequence: Synthetic polypeptide"
EVQLVQSGAEVKKPGESLKISCKGSGYTFTSYNMHWVRQMPGKGLEWMGDIYPGQGDTSYNQKFKGQVTISADKSISTVYLQWSSLKASDTAMYYCARVGGAFPMDYWGQGTTVTVSSASTKGPSVFPLAPCSRSTSESTAALGCLVKDYFPEPVTVSWNSGALTSGVHTFPAVLQSSGLYSLSSVVTVPSSSLGTKTYTCNVDHKPSNTKVDKRVESKYGPPCPPCPAPEFLGGPSVFLFPPKPKDTLMISRTPEVTCVVVDVSQEDPEVQFNWYVDGVEVHNAKTKPREEQFNSTYRVVSVLTVLHQDWLNGKEYKCKVSNKGLPSSIEKTISKAKGQPREPQVYTLPPSQEEMTKNQVSLTCLVKGFYPSDIAVEWESNGQPENNYKTTPPVLDSDGSFFLYSRLTVDKSRWQEGNVFSCSVMHEALHNHYTQKSLSLSLGK

SEQ ID NO: 83 - DNA, 1335 bp, synthetic construct
  misc_feature 1..1335: note = source = /note="Description of Artificial Sequence: Synthetic polynucleotide"
  source 1..1335: mol_type = other DNA
gaagttcaattggtacagtctggcgcagaagtaaagaaaccaggagagagtttgaaaatttcctgcaagggcagtgggtacacattcacgtcctacaatatgcactgggtgagacagatgccaggcaagggcctggagtggatgggagacatatacccaggccagggagacacaagctataatcagaaattcaaaggacaggtgacgatctccgcagacaaatccatatctacggtctacctccagtggtcctcacttaaagcctccgacaccgccatgtactattgcgctcgggtaggtggcgcgtttccaatggactattggggccaagggaccacagtaaccgtcagctcagcctctacaaagggcccctccgtctttccactcgcgccgtgctctcgctccacctcagagtcaactgccgctctgggttgcctggtcaaggactacttcccagagccggtgacagtgagctggaacagtggggccctgacatccggcgttcataccttccccgcagtcctccagtcctcaggcctgtattccctgagcagcgttgtcacagtgccctccagctctcttggcacgaaaacctacacatgcaacgttgatcataagccgtctaataccaaggtggataaaagagtggagagcaagtacggcccaccctgcccgccttgcccagctccggagttcctgggcggaccatccgttttcttgtttccacccaaacctaaagacactctgatgatttcccgaacccctgaagtgacttgcgttgtggtggacgtctcccaggaggacccagaagtgcaattcaactggtacgtggacggggtggaggtgcacaatgcaaaaaccaaaccaagggaggaacagtttaattcaacatatagggttgtgtctgtgctgacggttctgcatcaggactggctgaacggaaaggaatacaagtgcaaggtgtccaacaaaggactgccaagctctatcgagaaaacaatctctaaggccaagggacaacctagagagccccaagtttacaccctgccaccatcacaggaagagatgaccaaaaatcaggtgagcttgacatgcctggtgaagggcttctaccctagcgatattgcggttgagtgggagtcaaatggccagcctgagaacaactataagactactcctcccgtgctggactccgacgggagctttttcctgtattccaggcttacagtcgataagagcagatggcaagaggggaatgtgttttcctgctccgtgatgcacgaggctctccataaccattatactcagaaaagtctctctctgtcactgggcaaa

SEQ ID NO: 84 - protein, 118 aa, synthetic construct; identical to SEQ ID NO: 32
  REGION 1..118: note = source = /note="Description of Artificial Sequence: Synthetic polypeptide"

SEQ ID NO: 85 - DNA, 354 bp, synthetic construct
  misc_feature 1..354: note = source = /note="Description of Artificial Sequence: Synthetic polynucleotide"
  source 1..354: mol_type = other DNA
caggtgcaattggtgcagagcggagcagaggtcaaaaagcccggagcaagcgtgaaggtctcatgcaaagcaagcggatacacatttacatcatacaacatgcactgggtcaggcaggctccaggacagggactggagtggatcggggacatctaccctggacagggcgatactagctataatcagaagttcaaaggccgggccaccatgacagctgacaagtctactagtaccgtgtatatggaactgagctccctgcggtctgaagataccgcagtgtactattgcgccagagtcgggggggcatttcctatggattattgggggcaggggactctggtcactgtcagctca

SEQ ID NO: 86 - protein, 448 aa, synthetic construct
  REGION 1..448: note = source = /note="Description of Artificial Sequence: Synthetic polypeptide"
QVQLVQSGAEVKKPGASVKVSCKASGYTFTSYNMHWVRQAPGQGLEWIGDIYPGQGDTSYNQKFKGRATMTADKSTSTVYMELSSLRSEDTAVYYCARVGGAFPMDYWGQGTLVTVSSASTKGPSVFPLAPSSKSTSGGTAALGCLVKDYFPEPVTVSWNSGALTSGVHTFPAVLQSSGLYSLSSVVTVPSSSLGTQTYICNVNHKPSNTKVDKRVEPKSCDKTHTCPPCPAPELLGGPSVFLFPPKPKDTLMISRTPEVTCVVVAVSHEDPEVKFNWYVDGVEVHNAKTKPREEQYNSTYRVVSVLTVLHQDWLNGKEYKCKVSNKALAAPIEKTISKAKGQPREPQVYTLPPSREEMTKNQVSLTCLVKGFYPSDIAVEWESNGQPENNYKTTPPVLDSDGSFFLYSKLTVDKSRWQQGNVFSCSVMHEALHNHYTQKSLSLSPGK

SEQ ID NO: 87 - DNA, 1344 bp, synthetic construct
  misc_feature 1..1344: note = source = /note="Description of Artificial Sequence: Synthetic polynucleotide"
  source 1..1344: mol_type = other DNA
caggtgcaattggtgcagagcggagcagaggtcaaaaagcccggagcaagcgtgaaggtctcatgcaaagcaagcggatacacatttacatcatacaacatgcactgggtcaggcaggctccaggacagggactggagtggatcggggacatctaccctggacagggcgatactagctataatcagaagttcaaaggccgggccaccatgacagctgacaagtctactagtaccgtgtatatggaactgagctccctgcggtctgaagataccgcagtgtactattgcgccagagtcgggggggcatttcctatggattattgggggcaggggactctggtcactgtcagctcagctagcaccaagggccccagcgtgttccccctggcccccagcagcaagagcaccagcggcggcacagccgccctgggctgcctggtgaaggactacttccccgagcccgtgaccgtgtcctggaacagcggagccctgacctccggcgtgcacaccttccccgccgtgctgcagagcagcggcctgtacagcctgtccagcgtggtgacagtgcccagcagcagcctgggcacccagacctacatctgcaacgtgaaccacaagcccagcaacaccaaggtggacaagagagtggagcccaagagctgcgacaagacccacacctgccccccctgcccagccccagagctgctgggcggaccctccgtgttcctgttcccccccaagcccaaggacaccctgatgatcagcaggacccccgaggtgacctgcgtggtggtggccgtgagccacgaggacccagaggtgaagttcaactggtacgtggacggcgtggaggtgcacaacgccaagaccaagcccagagaggagcagtacaacagcacctacagggtggtgtccgtgctgaccgtgctgcaccaggactggctgaacggcaaggaatacaagtgcaaggtctccaacaaggccctggcagcccccatcgaaaagaccatcagcaaggccaagggccagccacgggagccccaggtgtacaccctgcccccctcccgggaggagatgaccaagaaccaggtgtccctgacctgtctggtgaagggcttctaccccagcgacatcgccgtggagtgggagagcaacggccagcccgagaacaactacaagaccacccccccagtgctggacagcgacggcagcttcttcctgtacagcaagctgaccgtggacaagtccaggtggcagcagggcaacgtgttcagctgcagcgtgatgcacgaggccctgcacaaccactacacccagaagagcctgagcctgtcccccggcaag

SEQ ID NO: 88 - protein, 111 aa, synthetic construct; identical to SEQ ID NO: 20
  REGION 1..111: note = source = /note="Description of Artificial Sequence: Synthetic polypeptide"

SEQ ID NO: 89 - DNA, 333 bp, synthetic construct
  misc_feature 1..333: note = source = /note="Description of Artificial Sequence: Synthetic polynucleotide"
  source 1..333: mol_type = other DNA
gacatcgtcctgacacagtctcctgacagcctggcagtgagcctgggcgaaagggcaaccattaattgtagagcttccgagtccgtcgagtactatggcactagtctgatgcagtggtaccagcagaagccagggcagccccctaaactgctgatctatgcagctagcaacgtggagtccggagtcccagaccggttctctggaagtgggtcaggaaccgattttaccctgacaattagctccctgcaggcagaagacgtggccgtctactattgtcagcagagccgcaaggacccaagcacattcggaggggggaccaaagtggaaatcaag

SEQ ID NO: 90 - protein, 218 aa, synthetic construct; identical to SEQ ID NO: 22
  REGION 1..218: note = source = /note="Description of Artificial Sequence: Synthetic polypeptide"

SEQ ID NO: 91 - DNA, 654 bp, synthetic construct
  misc_feature 1..654: note = source = /note="Description of Artificial Sequence: Synthetic polynucleotide"
  source 1..654: mol_type = other DNA
gacatcgtcctgacacagtctcctgacagcctggcagtgagcctgggcgaaagggcaaccattaattgtagagcttccgagtccgtcgagtactatggcactagtctgatgcagtggtaccagcagaagccagggcagccccctaaactgctgatctatgcagctagcaacgtggagtccggagtcccagaccggttctctggaagtgggtcaggaaccgattttaccctgacaattagctccctgcaggcagaagacgtggccgtctactattgtcagcagagccgcaaggacccaagcacattcggaggggggaccaaagtggaaatcaagcgtacggtggccgctcccagcgtgttcatcttcccccccagcgacgagcagctgaagagcggcaccgccagcgtggtgtgcctgctgaacaacttctacccccgggaggccaaggtgcagtggaaggtggacaacgccctgcagagcggcaacagccaggagagcgtcaccgagcaggacagcaaggactccacctacagcctgagcagcaccctgaccctgagcaaggccgactacgagaagcataaggtgtacgcctgcgaggtgacccaccagggcctgtccagccccgtgaccaagagcttcaacaggggcgagtgc

SEQ ID NO: 92 - protein, 118 aa, synthetic construct
  REGION 1..118: note = source = /note="Description of Artificial Sequence: Synthetic polypeptide"
QVQLVQSGAEVKKPGASVKVSCKASGYTFTSYNMHWVRQAPGQGLEWMGDIYPGQGDTSYNQKFKGRVTMTRDTSTSTVYMELSSLRSEDTAVYYCARVGGAFPMDYWGQGTTVTVSS

SEQ ID NO: 93 - DNA, 354 bp, synthetic construct
  misc_feature 1..354: note = source = /note="Description of Artificial Sequence: Synthetic polynucleotide"
  source 1..354: mol_type = other DNA
caggtgcagctggtgcagtctggcgccgaagtgaagaaaccaggcgccagcgtgaaggtgtcctgcaaggccagcggctacacctttaccagctacaacatgcactgggtgcgccaggcccctggacagggactggaatggatgggcgacatctaccccggccagggcgacacctcctacaaccagaaattcaagggcagagtgaccatgacccgggacaccagcacctccaccgtgtacatggaactgagcagcctgcggagcgaggacaccgccgtgtactactgtgctagagtgggcggagccttccccatggactattggggccagggcaccaccgtgaccgtgagctca

SEQ ID NO: 94 - protein, 448 aa, synthetic construct
  REGION 1..448: note = source = /note="Description of Artificial Sequence: Synthetic polypeptide"
QVQLVQSGAEVKKPGASVKVSCKASGYTFTSYNMHWVRQAPGQGLEWMGDIYPGQGDTSYNQKFKGRVTMTRDTSTSTVYMELSSLRSEDTAVYYCARVGGAFPMDYWGQGTTVTVSSASTKGPSVFPLAPSSKSTSGGTAALGCLVKDYFPEPVTVSWNSGALTSGVHTFPAVLQSSGLYSLSSVVTVPSSSLGTQTYICNVNHKPSNTKVDKRVEPKSCDKTHTCPPCPAPELLGGPSVFLFPPKPKDTLMISRTPEVTCVVVAVSHEDPEVKFNWYVDGVEVHNAKTKPREEQYNSTYRVVSVLTVLHQDWLNGKEYKCKVSNKALAAPIEKTISKAKGQPREPQVYTLPPSREEMTKNQVSLTCLVKGFYPSDIAVEWESNGQPENNYKTTPPVLDSDGSFFLYSKLTVDKSRWQQGNVFSCSVMHEALHNHYTQKSLSLSPGK

SEQ ID NO: 95 - DNA, 1344 bp, synthetic construct
  misc_feature 1..1344: note = source = /note="Description of Artificial Sequence: Synthetic polynucleotide"
  source 1..1344: mol_type = other DNA
caggtgcagctggtgcagtctggcgccgaagtgaagaaaccaggcgccagcgtgaaggtgtcctgcaaggccagcggctacacctttaccagctacaacatgcactgggtgcgccaggcccctggacagggactggaatggatgggcgacatctaccccggccagggcgacacctcctacaaccagaaattcaagggcagagtgaccatgacccgggacaccagcacctccaccgtgtacatggaactgagcagcctgcggagcgaggacaccgccgtgtactactgtgctagagtgggcggagccttccccatggactattggggccagggcaccaccgtgaccgtgagctcagctagcaccaagggccccagcgtgttccccctggcccccagcagcaagagcaccagcggcggcacagccgccctgggctgcctggtgaaggactacttccccgagcccgtgaccgtgtcctggaacagcggagccctgacctccggcgtgcacaccttccccgccgtgctgcagagcagcggcctgtacagcctgtccagcgtggtgacagtgcccagcagcagcctgggcacccagacctacatctgcaacgtgaaccacaagcccagcaacaccaaggtggacaagagagtggagcccaagagctgcgacaagacccacacctgccccccctgcccagccccagagctgctgggcggaccctccgtgttcctgttcccccccaagcccaaggacaccctgatgatcagcaggacccccgaggtgacctgcgtggtggtggccgtgagccacgaggacccagaggtgaagttcaactggtacgtggacggcgtggaggtgcacaacgccaagaccaagcccagagaggagcagtacaacagcacctacagggtggtgtccgtgctgaccgtgctgcaccaggactggctgaacggcaaggaatacaagtgcaaggtctccaacaaggccctggcagcccccatcgaaaagaccatcagcaaggccaagggccagccacgggagccccaggtgtacaccctgcccccctcccgggaggagatgaccaagaaccaggtgtccctgacctgtctggtgaagggcttctaccccagcgacatcgccgtggagtgggagagcaacggccagcccgagaacaactacaagaccacccccccagtgctggacagcgacggcagcttcttcctgtacagcaagctgaccgtggacaagtccaggtggcagcagggcaacgtgttcagctgcagcgtgatgcacgaggccctgcacaaccactacacccagaagagcctgagcctgtcccccggcaag

SEQ ID NO: 96 - protein, 111 aa, synthetic construct
  REGION 1..111: note = source = /note="Description of Artificial Sequence: Synthetic polypeptide"
AIRLTQSPSSFSASTGDRVTITCRASESVEYYGTSLMQWYQQKPGKAPKLLIYAASNVESGVPSRFSGSGSGTDFTLTISSLQSEDFATYYCQQSRKDPSTFGGGTKVEIK

SEQ ID NO: 97 - DNA, 333 bp, synthetic construct
  misc_feature 1..333: note = source = /note="Description of Artificial Sequence: Synthetic polynucleotide"
  source 1..333: mol_type = other DNA
gccatcagactgacccagagccccagctcctttagcgccagcaccggcgacagagtgaccatcacctgtagagccagcgagagcgtggaatattacggcaccagcctgatgcagtggtatcagcagaagcccggcaaggcccccaagctgctgatctacgccgccagcaatgtggaaagcggcgtgcccagcagattcagcggctctggcagcggcaccgacttcaccctgacaatcagcagcctgcagagcgaggacttcgccacctactactgccagcagagccggaaggaccccagcacatttggcggaggcaccaaggtggaaatcaag

SEQ ID NO: 98 - protein, 218 aa, synthetic construct
  REGION 1..218: note = source = /note="Description of Artificial Sequence: Synthetic polypeptide"
AIRLTQSPSSFSASTGDRVTITCRASESVEYYGTSLMQWYQQKPGKAPKLLIYAASNVESGVPSRFSGSGSGTDFTLTISSLQSEDFATYYCQQSRKDPSTFGGGTKVEIKRTVAAPSVFIFPPSDEQLKSGTASVVCLLNNFYPREAKVQWKVDNALQSGNSQESVTEQDSKDSTYSLSSTLTLSKADYEKHKVYACEVTHQGLSSPVTKSFNRGEC

SEQ ID NO: 99 - DNA, 654 bp, synthetic construct
  misc_feature 1..654: note = source = /note="Description of Artificial Sequence: Synthetic polynucleotide"
  source 1..654: mol_type = other DNA
gccatcagactgacccagagccccagctcctttagcgccagcaccggcgacagagtgaccatcacctgtagagccagcgagagcgtggaatattacggcaccagcctgatgcagtggtatcagcagaagcccggcaaggcccccaagctgctgatctacgccgccagcaatgtggaaagcggcgtgcccagcagattcagcggctctggcagcggcaccgacttcaccctgacaatcagcagcctgcagagcgaggacttcgccacctactactgccagcagagccggaaggaccccagcacatttggcggaggcaccaaggtggaaatcaagcgtacggtggccgctcccagcgtgttcatcttcccccccagcgacgagcagctgaagagcggcaccgccagcgtggtgtgcctgctgaacaacttctacccccgggaggccaaggtgcagtggaaggtggacaacgccctgcagagcggcaacagccaggagagcgtcaccgagcaggacagcaaggactccacctacagcctgagcagcaccctgaccctgagcaaggccgactacgagaagcataaggtgtacgcctgcgaggtgacccaccagggcctgtccagccccgtgaccaagagcttcaacaggggcgagtgc

SEQ ID NO: 100 - protein, 118 aa, synthetic construct
  REGION 1..118: note = source = /note="Description of Artificial Sequence: Synthetic polypeptide"
QVQLVQSGAEVKKPGESLKISCKGSGYTFTSYNMHWVRQMPGKGLEWMGDIYPGNGDTSYNQKFKGQVTISADKSISTVYLQWSSLKASDTAMYYCARVGGAFPMDYWGQGTTVTVSS

SEQ ID NO: 101 - DNA, 354 bp, synthetic construct
  misc_feature 1..354: note = source = /note="Description of Artificial Sequence: Synthetic polynucleotide"
  source 1..354: mol_type = other DNA
caggtgcaattggtacagtctggcgcagaagtaaagaaaccaggagagagtttgaaaatttcctgcaagggcagtgggtacacattcacgtcctacaatatgcactgggtgagacagatgccaggcaagggcctggagtggatgggagacatatacccaggcaatggagacacaagctataatcagaaattcaaaggacaggtgacgatctccgcagacaaatccatatctacggtctacctccagtggtcctcacttaaagcctccgacaccgccatgtactattgcgctcgggtaggtggcgcgtttccaatggactattggggccaagggaccacagtaaccgtcagctca

SEQ ID NO: 102 - protein, 448 aa, synthetic construct
  REGION 1..448: note = source = /note="Description of Artificial Sequence: Synthetic polypeptide"
QVQLVQSGAEVKKPGESLKISCKGSGYTFTSYNMHWVRQMPGKGLEWMGDIYPGNGDTSYNQKFKGQVTISADKSISTVYLQWSSLKASDTAMYYCARVGGAFPMDYWGQGTTVTVSSASTKGPSVFPLAPSSKSTSGGTAALGCLVKDYFPEPVTVSWNSGALTSGVHTFPAVLQSSGLYSLSSVVTVPSSSLGTQTYICNVNHKPSNTKVDKRVEPKSCDKTHTCPPCPAPELLGGPSVFLFPPKPKDTLMISRTPEVTCVVVAVSHEDPEVKFNWYVDGVEVHNAKTKPREEQYNSTYRVVSVLTVLHQDWLNGKEYKCKVSNKALAAPIEKTISKAKGQPREPQVYTLPPSREEMTKNQVSLTCLVKGFYPSDIAVEWESNGQPENNYKTTPPVLDSDGSFFLYSKLTVDKSRWQQGNVFSCSVMHEALHNHYTQKSLSLSPGK

SEQ ID NO: 103 - DNA, 1344 bp, synthetic construct
  misc_feature 1..1344: note = source = /note="Description of Artificial Sequence: Synthetic polynucleotide"
  source 1..1344: mol_type = other DNA
caggtgcaattggtacagtctggcgcagaagtaaagaaaccaggagagagtttgaaaatttcctgcaagggcagtgggtacacattcacgtcctacaatatgcactgggtgagacagatgccaggcaagggcctggagtggatgggagacatatacccaggcaatggagacacaagctataatcagaaattcaaaggacaggtgacgatctccgcagacaaatccatatctacggtctacctccagtggtcctcacttaaagcctccgacaccgccatgtactattgcgctcgggtaggtggcgcgtttccaatggactattggggccaagggaccacagtaaccgtcagctcagctagcaccaagggccccagcgtgttccccctggcccccagcagcaagagcaccagcggcggcacagccgccctgggctgcctggtgaaggactacttccccgagcccgtgaccgtgtcctggaacagcggagccctgacctccggcgtgcacaccttccccgccgtgctgcagagcagcggcctgtacagcctgtccagcgtggtgacagtgcccagcagcagcctgggcacccagacctacatctgcaacgtgaaccacaagcccagcaacaccaaggtggacaagagagtggagcccaagagctgcgacaagacccacacctgccccccctgcccagccccagagctgctgggcggaccctccgtgttcctgttcccccccaagcccaaggacaccctgatgatcagcaggacccccgaggtgacctgcgtggtggtggccgtgagccacgaggacccagaggtgaagttcaactggtacgtggacggcgtggaggtgcacaacgccaagaccaagcccagagaggagcagtacaacagcacctacagggtggtgtccgtgctgaccgtgctgcaccaggactggctgaacggcaaggaatacaagtgcaaggtctccaacaaggccctggcagcccccatcgaaaagaccatcagcaaggccaagggccagccacgggagccccaggtgtacaccctgcccccctcccgggaggagatgaccaagaaccaggtgtccctgacctgtctggtgaagggcttctaccccagcgacatcgccgtggagtgggagagcaacggccagcccgagaacaactacaagaccacccccccagtgctggacagcgacggcagcttcttcctgtacagcaagctgaccgtggacaagtccaggtggcagcagggcaacgtgttcagctgcagcgtgatgcacgaggccctgcacaaccactacacccagaagagcctgagcctgtcccccggcaag

SEQ ID NO: 104 - protein, 111 aa, synthetic construct; identical to SEQ ID NO: 64
  REGION 1..111: note = source = /note="Description of Artificial Sequence: Synthetic polypeptide"

SEQ ID NO: 105 - DNA, 333 bp, synthetic construct
  misc_feature 1..333: note = source = /note="Description of Artificial Sequence: Synthetic polynucleotide"
  source 1..333: mol_type = other DNA
gcaatacagttgacacagagtccttcaagtttgtccgcttccgttggcgaccgagtgacaatcacctgtagagcatccgagtcagtggagtattatggcactagcctgatgcagtggtatcagcaaaagccagggaaagccccaaagctgctgatatatgccgcgagtaacgtcgagtcaggggtgccatcaagattctccggttccgggtccggaaccgacttcacactgaccatctcttcccttcagccagaggacttcgctacgtacttttgccagcagtcacggaaagatccctctactttcggaggtgggacaaaagtcgaaattaaa

SEQ ID NO: 106 - protein, 218 aa, synthetic construct; identical to SEQ ID NO: 66
  REGION 1..218: note = source = /note="Description of Artificial Sequence: Synthetic polypeptide"

SEQ ID NO: 107 - DNA, 654 bp, synthetic construct
  misc_feature 1..654: note = source = /note="Description of Artificial Sequence: Synthetic polynucleotide"
  source 1..654: mol_type = other DNA
gcaatacagttgacacagagtccttcaagtttgtccgcttccgttggcgaccgagtgacaatcacctgtagagcatccgagtcagtggagtattatggcactagcctgatgcagtggtatcagcaaaagccagggaaagccccaaagctgctgatatatgccgcgagtaacgtcgagtcaggggtgccatcaagattctccggttccgggtccggaaccgacttcacactgaccatctcttcccttcagccagaggacttcgctacgtacttttgccagcagtcacggaaagatccctctactttcggaggtgggacaaaagtcgaaattaaacgtacggtggccgctcccagcgtgttcatcttcccccccagcgacgagcagctgaagagcggcaccgccagcgtggtgtgcctgctgaacaacttctacccccgggaggccaaggtgcagtggaaggtggacaacgccctgcagagcggcaacagccaggagagcgtcaccgagcaggacagcaaggactccacctacagcctgagcagcaccctgaccctgagcaaggccgactacgagaagcataaggtgtacgcctgcgaggtgacccaccagggcctgtccagccccgtgaccaagagcttcaacaggggcgagtgc

SEQ ID NO: 108 - protein, 327 aa, Homo sapiens
ASTKGPSVFPLAPCSRSTSESTAALGCLVKDYFPEPVTVSWNSGALTSGVHTFPAVLQSSGLYSLSSVVTVPSSSLGTKTYTCNVDHKPSNTKVDKRVESKYGPPCPPCPAPEFLGGPSVFLFPPKPKDTLMISRTPEVTCVVVDVSQEDPEVQFNWYVDGVEVHNAKTKPREEQFNSTYRVVSVLTVLHQDWLNGKEYKCKVSNKGLPSSIEKTISKAKGQPREPQVYTLPPSQEEMTKNQVSLTCLVKGFYPSDIAVEWESNGQPENNYKTTPPVLDSDGSFFLYSRLTVDKSRWQEGNVFSCSVMHEALHNHYTQKSLSLSLGK

SEQ ID NO: 109 - protein, 107 aa, Homo sapiens [sequence omitted]

SEQ ID NO: 110 - protein, 326 aa, Homo sapiens
ASTKGPSVFPLAPCSRSTSESTAALGCLVKDYFPEPVTVSWNSGALTSGVHTFPAVLQSSGLYSLSSVVTVPSSSLGTKTYTCNVDHKPSNTKVDKRVESKYGPPCPPCPAPEFLGGPSVFLFPPKPKDTLMISRTPEVTCVVVDVSQEDPEVQFNWYVDGVEVHNAKTKPREEQFNSTYRVVSVLTVLHQDWLNGKEYKCKVSNKGLPSSIEKTISKAKGQPREPQVYTLPPSQEEMTKNQVSLTCLVKGFYPSDIAVEWESNGQPENNYKTTPPVLDSDGSFFLYSRLTVDKSRWQEGNVFSCSVMHEALHNHYTQKSLSLSLG

SEQ ID NO: 111 - protein, 330 aa, Homo sapiens
ASTKGPSVFPLAPSSKSTSGGTAALGCLVKDYFPEPVTVSWNSGALTSGVHTFPAVLQSSGLYSLSSVVTVPSSSLGTQTYICNVNHKPSNTKVDKRVEPKSCDKTHTCPPCPAPELLGGPSVFLFPPKPKDTLMISRTPEVTCVVVDVSHEDPEVKFNWYVDGVEVHNAKTKPREEQYNSTYRVVSVLTVLHQDWLNGKEYKCKVSNKALPAPIEKTISKAKGQPREPQVYTLPPSREEMTKNQVSLTCLVKGFYPSDIAVEWESNGQPENNYKTTPPVLDSDGSFFLYSKLTVDKSRWQQGNVFSCSVMHEALHNHYTQKSLSLSPGK

SEQ ID NO: 112 - protein, 330 aa, Homo sapiens
ASTKGPSVFPLAPSSKSTSGGTAALGCLVKDYFPEPVTVSWNSGALTSGVHTFPAVLQSSGLYSLSSVVTVPSSSLGTQTYICNVNHKPSNTKVDKRVEPKSCDKTHTCPPCPAPELLGGPSVFLFPPKPKDTLMISRTPEVTCVVVDVSHEDPEVKFNWYVDGVEVHNAKTKPREEQYASTYRVVSVLTVLHQDWLNGKEYKCKVSNKALPAPIEKTISKAKGQPREPQVYTLPPSREEMTKNQVSLTCLVKGFYPSDIAVEWESNGQPENNYKTTPPVLDSDGSFFLYSKLTVDKSRWQQGNVFSCSVMHEALHNHYTQKSLSLSPGK

SEQ ID NO: 113 - protein, 330 aa, Homo sapiens
ASTKGPSVFPLAPSSKSTSGGTAALGCLVKDYFPEPVTVSWNSGALTSGVHTFPAVLQSSGLYSLSSVVTVPSSSLGTQTYICNVNHKPSNTKVDKRVEPKSCDKTHTCPPCPAPELLGGPSVFLFPPKPKDTLMISRTPEVTCVVVAVSHEDPEVKFNWYVDGVEVHNAKTKPREEQYNSTYRVVSVLTVLHQDWLNGKEYKCKVSNKALAAPIEKTISKAKGQPREPQVYTLPPSREEMTKNQVSLTCLVKGFYPSDIAVEWESNGQPENNYKTTPPVLDSDGSFFLYSKLTVDKSRWQQGNVFSCSVMHEALHNHYTQKSLSLSPGK

SEQ ID NO: 114 - protein, 330 aa, Homo sapiens
ASTKGPSVFPLAPSSKSTSGGTAALGCLVKDYFPEPVTVSWNSGALTSGVHTFPAVLQSSGLYSLSSVVTVPSSSLGTQTYICNVNHKPSNTKVDKRVEPKSCDKTHTCPPCPAPEAAGGPSVFLFPPKPKDTLMISRTPEVTCVVVDVSHEDPEVKFNWYVDGVEVHNAKTKPREEQYNSTYRVVSVLTVLHQDWLNGKEYKCKVSNKALPAPIEKTISKAKGQPREPQVYTLPPSREEMTKNQVSLTCLVKGFYPSDIAVEWESNGQPENNYKTTPPVLDSDGSFFLYSKLTVDKSRWQQGNVFSCSVMHEALHNHYTQKSLSLSPGK

SEQ ID NO: 115 - DNA, 354 bp, synthetic construct
  misc_feature 1..354: note = source = /note="Description of Artificial Sequence: Synthetic polynucleotide"
  source 1..354: mol_type = other DNA
caggtccagctggtccagagcggagcagaggtcaaaaagcccggagcaagcgtgaaggtctcatgcaaagcaagcggatacacatttacatcatacaacatgcactggatcaggcaggctccaggacagggactggagtggatcggggacatctaccctggaaacggcgatactagctataatcagaagttcaaaggccgggccaccctgacagctgacaagtctactagtaccgtgtatatggagctgagctccctgcggtctgaagataccgcagtgtactattgcgccagagtcgggggggcatttcctatggattattgggggcaggggactctggtcactgtctcctcc

SEQ ID NO: 116 - protein, 445 aa, synthetic construct
  REGION 1..445: note = source = /note="Description of Artificial Sequence: Synthetic polypeptide"
QVQLVQSGAEVKKPGASVKVSCKASGYTFTSYNMHWIRQAPGQGLEWIGDIYPGNGDTSYNQKFKGRATLTADKSTSTVYMELSSLRSEDTAVYYCARVGGAFPMDYWGQGTLVTVSSASTKGPSVFPLAPCSRSTSESTAALGCLVKDYFPEPVTVSWNSGALTSGVHTFPAVLQSSGLYSLSSVVTVPSSSLGTKTYTCNVDHKPSNTKVDKRVESKYGPPCPPCPAPEFLGGPSVFLFPPKPKDTLMISRTPEVTCVVVDVSQEDPEVQFNWYVDGVEVHNAKTKPREEQFNSTYRVVSVLTVLHQDWLNGKEYKCKVSNKGLPSSIEKTISKAKGQPREPQVYTLPPSQEEMTKNQVSLTCLVKGFYPSDIAVEWESNGQPENNYKTTPPVLDSDGSFFLYSRLTVDKSRWQEGNVFSCSVMHEALHNHYTQKSLSLSLGK

SEQ ID NO: 117 - DNA, 1335 bp, synthetic construct
  misc_feature 1..1335: note = source = /note="Description of Artificial Sequence: Synthetic polynucleotide"
  source 1..1335: mol_type = other DNA
caggtccagctggtccagagcggagcagaggtcaaaaagcccggagcaagcgtgaaggtctcatgcaaagcaagcggatacacatttacatcatacaacatgcactggatcaggcaggctccaggacagggactggagtggatcggggacatctaccctggaaacggcgatactagctataatcagaagttcaaaggccgggccaccctgacagctgacaagtctactagtaccgtgtatatggagctgagctccctgcggtctgaagataccgcagtgtactattgcgccagagtcgggggggcatttcctatggattattgggggcaggggactctggtcactgtctcctccgctagcaccaagggcccatccgtcttccccctggcgccctgctccaggagcacctccgagagcacagccgccctgggctgcctggtcaaggactacttccccgaaccggtgacggtgtcgtggaactcaggcgccctgaccagcggcgtgcacaccttcccggctgtcctacagtcctcaggactctactccctcagcagcgtggtgaccgtgccctccagcagcttgggcacgaagacctacacctgcaacgtagatcacaagcccagcaacaccaaggtggacaagagagttgagtccaaatatggtcccccatgcccaccatgcccagcacctgagttcctggggggaccatcagtcttcctgttccccccaaaacccaaggacactctcatgatctcccggacccctgaggtcacgtgcgtggtggtggacgtgagccaggaagaccccgaggtccagttcaactggtacgtggatggcgtggaggtgcataatgccaagacaaagccgcgggaggagcagttcaacagcacgtaccgtgtggtcagcgtcctcaccgtcctgcaccaggactggctgaacggcaaggagtacaagtgcaaggtctccaacaaaggcctcccgtcctccatcgagaaaaccatctccaaagccaaagggcagccccgagagccacaggtgtacaccctgcccccatcccaggaggagatgaccaagaaccaggtcagcctgacctgcctggtcaaaggcttctaccccagcgacatcgccgtggagtgggagagcaatgggcagccggagaacaactacaagaccacgcctcccgtgctggactccgacggctccttcttcctctacagcaggctaaccgtggacaagagcaggtggcaggaggggaatgtcttctcatgctccgtgatgcatgaggctctgcacaaccactacacacagaagagcctctccctgtctctgggtaaa

SEQ ID NO: 118 - DNA, 333 bp, synthetic construct; identical to SEQ ID NO: 89
  misc_feature 1..333: note = source = /note="Description of Artificial Sequence: Synthetic polynucleotide"
  source 1..333: mol_type = other DNA

SEQ ID NO: 119 - DNA, 654 bp, synthetic construct
  misc_feature 1..654: note = source = /note="Description of Artificial Sequence: Synthetic polynucleotide"
  source 1..654: mol_type = other DNA
gacatcgtcctgacacagtctcctgacagcctggcagtgagcctgggcgaaagggcaaccattaattgtagagcttccgagtccgtcgagtactatggcactagtctgatgcagtggtaccagcagaagccagggcagccccctaaactgctgatctatgcagctagcaacgtggagtccggagtcccagaccggttctctggaagtgggtcaggaaccgattttaccctgacaattagctccctgcaggcagaagacgtggccgtctactattgtcagcagagccgcaaggacccaagcacattcggaggggggaccaaagtggaaatcaagcggactgttgctgcaccatctgtcttcatcttcccgccatctgatgagcagttgaaatctggaactgcctctgttgtgtgcctgctgaataacttctatcccagagaggccaaagtacagtggaaggtggataacgccctccaatcgggtaactcccaggagagtgtcacagagcaggacagcaaggacagcacctacagcctcagcagcaccctgacgctgagcaaagcagactacgagaaacacaaagtctacgcctgcgaagtcacccatcagggcctgagttcaccggtgacaaagagcttcaacaggggagagtgt

SEQ ID NO: 120 - DNA, 354 bp, synthetic construct
  misc_feature 1..354: note = source = /note="Description of Artificial Sequence: Synthetic polynucleotide"
  source 1..354: mol_type = other DNA
caggtccagctggtccagagcggagcagaggtcaaaaagcccggagcaagcgtgaaggtctcatgcaaagcaagcggatacacatttacatcatacaacatgcactgggtcaggcaggctccaggacagggactggagtggatcggggacatctaccctggaaacggcgatactagctataatcagaagttcaaaggccgggccaccatgacagctgacaagtctactagtaccgtgtatatggagctgagctccctgcggtctgaagataccgcagtgtactattgcgccagagtcgggggggcatttcctatggattattgggggcaggggactctggtcactgtctcctcc

SEQ ID NO: 121 - protein, 445 aa, synthetic construct
  REGION 1..445: note = source = /note="Description of Artificial Sequence: Synthetic polypeptide"
QVQLVQSGAEVKKPGASVKVSCKASGYTFTSYNMHWVRQAPGQGLEWIGDIYPGNGDTSYNQKFKGRATMTADKSTSTVYMELSSLRSEDTAVYYCARVGGAFPMDYWGQGTLVTVSSASTKGPSVFPLAPCSRSTSESTAALGCLVKDYFPEPVTVSWNSGALTSGVHTFPAVLQSSGLYSLSSVVTVPSSSLGTKTYTCNVDHKPSNTKVDKRVESKYGPPCPPCPAPEFLGGPSVFLFPPKPKDTLMISRTPEVTCVVVDVSQEDPEVQFNWYVDGVEVHNAKTKPREEQFNSTYRVVSVLTVLHQDWLNGKEYKCKVSNKGLPSSIEKTISKAKGQPREPQVYTLPPSQEEMTKNQVSLTCLVKGFYPSDIAVEWESNGQPENNYKTTPPVLDSDGSFFLYSRLTVDKSRWQEGNVFSCSVMHEALHNHYTQKSLSLSLGK

SEQ ID NO: 122 - DNA, 1335 bp, synthetic construct
  misc_feature 1..1335: note = source = /note="Description of Artificial Sequence: Synthetic polynucleotide"
  source 1..1335: mol_type = other DNA
caggtccagctggtccagagcggagcagaggtcaaaaagcccggagcaagcgtgaaggtctcatgcaaagcaagcggatacacatttacatcatacaacatgcactgggtcaggcaggctccaggacagggactggagtggatcggggacatctaccctggaaacggcgatactagctataatcagaagttcaaaggccgggccaccatgacagctgacaagtctactagtaccgtgtatatggagctgagctccctgcggtctgaagataccgcagtgtactattgcgccagagtcgggggggcatttcctatggattattgggggcaggggactctggtcactgtctcctccgctagcaccaagggcccatccgtcttccccctggcgccctgctccaggagcacctccgagagcacagccgccctgggctgcctggtcaaggactacttccccgaaccggtgacggtgtcgtggaactcaggcgccctgaccagcggcgtgcacaccttcccggctgtcctacagtcctcaggactctactccctcagcagcgtggtgaccgtgccctccagcagcttgggcacgaagacctacacctgcaacgtagatcacaagcccagcaacaccaaggtggacaagagagttgagtccaaatatggtcccccatgcccaccatgcccagcacctgagttcctggggggaccatcagtcttcctgttccccccaaaacccaaggacactctcatgatctcccggacccctgaggtcacgtgcgtggtggtggacgtgagccaggaagaccccgaggtccagttcaactggtacgtggatggcgtggaggtgcataatgccaagacaaagccgcgggaggagcagttcaacagcacgtaccgtgtggtcagcgtcctcaccgtcctgcaccaggactggctgaacggcaaggagtacaagtgcaaggtctccaacaaaggcctcccgtcctccatcgagaaaaccatctccaaagccaaagggcagccccgagagccacaggtgtacaccctgcccccatcccaggaggagatgaccaagaaccaggtcagcctgacctgcctggtcaaaggcttctaccccagcgacatcgccgtggagtgggagagcaatgggcagccggagaacaactacaagaccacgcctcccgtgctggactccgacggctccttcttcctctacagcaggctaaccgtggacaagagcaggtggcaggaggggaatgtcttctcatgctccgtgatgcatgaggctctgcacaaccactacacacagaagagcctctccctgtctctgggtaaa

SEQ ID NO: 123 - DNA, 333 bp, synthetic construct
  misc_feature 1..333: note = source = /note="Description of Artificial Sequence: Synthetic polynucleotide"
  source 1..333: mol_type = other DNA
gacatcgtcctgacacagtctcctgacagcctggcagtgagcctgggcgaaagggcaaccattaattgtagagcttccgagtccgtcgagtactatggcactagtctgatgcagtggtaccagcagaagccagggcagccccctaaactgctgatctatgcagctagcaacgtggagtccggagtcccagaccggttctctggaagtgggtcaggaaccgattttaccctgacaattagctccctgcaggcagaagacgtggccgtctacttttgtcagcagagccgcaaggacccaagcacattcggaggggggaccaaagtggaaatcaag

SEQ ID NO: 124 - DNA, 654 bp, synthetic construct
  misc_feature 1..654: note = source = /note="Description of Artificial Sequence: Synthetic polynucleotide"
  source 1..654: mol_type = other DNA
gacatcgtcctgacacagtctcctgacagcctggcagtgagcctgggcgaaagggcaaccattaattgtagagcttccgagtccgtcgagtactatggcactagtctgatgcagtggtaccagcagaagccagggcagccccctaaactgctgatctatgcagctagcaacgtggagtccggagtcccagaccggttctctggaagtgggtcaggaaccgattttaccctgacaattagctccctgcaggcagaagacgtggccgtctacttttgtcagcagagccgcaaggacccaagcacattcggaggggggaccaaagtggaaatcaagcggactgttgctgcaccatctgtcttcatcttcccgccatctgatgagcagttgaaatctggaactgcctctgttgtgtgcctgctgaataacttctatcccagagaggccaaagtacagtggaaggtggataacgccctccaatcgggtaactcccaggagagtgtcacagagcaggacagcaaggacagcacctacagcctcagcagcaccctgacgctgagcaaagcagactacgagaaacacaaagtctacgcctgcgaagtcacccatcagggcctgagttcaccggtgacaaagagcttcaacaggggagagtgt

SEQ ID NO: 125 - DNA, 333 bp, synthetic construct; identical to SEQ ID NO: 105
  misc_feature 1..333: note = source = /note="Description of Artificial Sequence: Synthetic polynucleotide"
  source 1..333: mol_type = other DNA

SEQ ID NO: 126 - DNA, 654 bp, synthetic construct
  misc_feature 1..654: note = source = /note="Description of Artificial Sequence: Synthetic polynucleotide"
  source 1..654: mol_type = other DNA
gcaatacagttgacacagagtccttcaagtttgtccgcttccgttggcgaccgagtgacaatcacctgtagagcatccgagtcagtggagtattatggcactagcctgatgcagtggtatcagcaaaagccagggaaagccccaaagctgctgatatatgccgcgagtaacgtcgagtcaggggtgccatcaagattctccggttccgggtccggaaccgacttcacactgaccatctcttcccttcagccagaggacttcgctacgtacttttgccagcagtcacggaaagatccctctactttcggaggtgggacaaaagtcgaaattaaacgtacggtggcagctccgtctgttttcatctttccacctagcgacgagcaactcaaaagtggtacagcatccgtggtttgtctgctgaacaatttttaccccagggaggctaaggtccagtggaaagtcgataacgctcttcagtctggcaacagtcaggagagcgtcacagagcaggactctaaggatagcacttatagtctgtcctccacgctgacactgtctaaagcggattatgagaagcacaaggtttacgcctgtgaggtaacgcaccaaggactctcctccccagttaccaaatctttcaacagaggagaatgt

SEQ ID NO: 127 - DNA, 333 bp, synthetic construct
  misc_feature 1..333: note = source = /note="Description of Artificial Sequence: Synthetic polynucleotide"
  source 1..333: mol_type = other DNA
gagattgttcttacgcaaagtcccgccacacttagtttgtcaccaggagagcgcgccaccctgagctgcagagcttcagagagtgtggaatactacggcacatccctgatgcagtggtatcagcagaaaccaggacaggctcctcggctgctgatctacgcagccagcaacgtcgagtccggcattccagccagattttctgggtcaggatctggaactgactttacactgacaatctccagcctggaacccgaggacattgctgtgtatttttgtcaacagtcccggaaggaccccagtacctttggaggtggaaccaaggtagagataaag

SEQ ID NO: 128 - DNA, 654 bp, synthetic construct
  misc_feature 1..654: note = source = /note="Description of Artificial Sequence: Synthetic polynucleotide"
  source 1..654: mol_type = other DNA
gagattgttcttacgcaaagtcccgccacacttagtttgtcaccaggagagcgcgccaccctgagctgcagagcttcagagagtgtggaatactacggcacatccctgatgcagtggtatcagcagaaaccaggacaggctcctcggctgctgatctacgcagccagcaacgtcgagtccggcattccagccagattttctgggtcaggatctggaactgactttacactgacaatctccagcctggaacccgaggacattgctgtgtatttttgtcaacagtcccggaaggaccccagtacctttggaggtggaaccaaggtagagataaagcgtacggtggcagctccgtctgttttcatctttccacctagcgacgagcaactcaaaagtggtacagcatccgtggtttgtctgctgaacaatttttaccccagggaggctaaggtccagtggaaagtcgataacgctcttcagtctggcaacagtcaggagagcgtcacagagcaggactctaaggatagcacttatagtctgtcctccacgctgacactgtctaaagcggattatgagaagcacaaggtttacgcctgtgaggtaacgcaccaaggactctcctccccagttaccaaatctttcaacagaggagaatgt

SEQ ID NO: 129 - protein, 301 aa, Homo sapiens
MFSHLPFDCVLLLLLLLLTRSSEVEYRAEVGQNAYLPCFYTPAAPGNLVPVCWGKGACPVFECGNVVLRTDERDVNYWTSRYWLNGDFRKGDVSLTIENVTLADSGIYCCRIQIPGIMNDEKFNLKLVIKPAKVTPAPTRQRDFTAAFPRMLTTRGHGPAETQTLGSLPDINLTQISTLANELRDSRLANDLRDSGATIRIGIYIGAGICAGLALALIFGALIFKWYSHSKEKIQNLSLISLANLPPSGLANAVAEGIRSEENIYTIEENVYEVEEPNEYYCYVSSRQQPSQPLGCRFAMP

SEQ ID NO: 130 - protein, 135 aa, Homo sapiens
METDTLLLWVLLLWVPGSTGSEVEYRAEVGQNAYLPCFYTPAAPGNLVPVCWGKGACPVFECGNVVLRTDERDVNYWTSRYWLNGDFRKGDVSLTIENVTLADSGIYCCRIQIPGIMNDEKFNLKLVIKHHHHHH

SEQ ID NO: 131 - protein, 225 aa, synthetic construct
  REGION 1..225: note = source = /note="Description of Artificial Sequence: Synthetic polypeptide"
QVQLVQSGAEVKKPGASVKVSCKASGYTFTSYNMHWVRQAPGQGLEWIGDIYPGQGDTSYNQKFKGRATMTADKSTSTVYMELSSLRSEDTAVYYCARVGGAFPMDYWGQGTLVTVSSASTKGPSVFPLAPSSKSTSGGTAALGCLVKDYFPEPVTVSWNSGALTSGVHTFPAVLQSSGLYSLSSVVTVPSSSLGTQTYICNVNHKPSNTKVDKRVEPKSCDKTH

SEQ ID NO: 132 - protein, 218 aa, synthetic construct; identical to SEQ ID NO: 22
  REGION 1..218: note = source = /note="Description of Artificial Sequence: Synthetic polypeptide"

SEQ ID NO: 133 - protein, 6 aa, synthetic construct
  REGION 1..6: note = source = /note="Description of Artificial Sequence: Synthetic 6xHis tag"
HHHHHH

SEQ ID NO: 134 - protein, 98 aa, synthetic construct
  REGION 1..98: note = source = /note="Description of Artificial Sequence: Synthetic polypeptide"
QAYLQQSGAELVRPGASVKMSCKASGYTFTSYNMHWVKQTPRQGLEWIGAIYPGNGDTSYNQKFKGKATLTVDKSSSTAYMQLSSLTSEDSAVYFCAR

SEQ ID NO: 135 - protein, 111 aa, synthetic construct
  REGION 1..111: note = source = /note="Description of Artificial Sequence: Synthetic polypeptide"
DIVLTQSPASLAVSLGQRATISCRASESVEYYGTSLMQWYQQKPGQPPKLLIYAASNVESGVPARFSGSGSGTDFSLNIHPVEEDDIAMYFCQQSRKVPSTFGGGTKLEIK

SEQ ID NO: 136 - protein, 6 aa, synthetic construct
  REGION 1..6: note = source = /note="Description of Artificial Sequence: Synthetic peptide"
GACPVF

SEQ ID NO: 137 - protein, 9 aa, synthetic construct
  REGION 1..9: note = source = /note="Description of Artificial Sequence: Synthetic peptide"
NDEKFNLKL

SEQ ID NO: 138 - protein, 4 aa, synthetic construct
  REGION 1..4: note = source = /note="Description of Artificial Sequence: Synthetic peptide"
IMND

SEQ ID NO: 139 - protein, 114 aa, Homo sapiens
SEVEYRAEVGQNAYLPCFYTPAAPGNLVPVCWGKGACPVFECGNVVLRTDERDVNYWTSRYWLNGDFRKGDVSLTIENVTLADSGIYCCRIQIPGIMNDEKFNLKLVIKPAKVT

SEQ ID NO: 140 - protein, 21 aa, Homo sapiens
TPAAPGNLVPVCWGKGACPVF

SEQ ID NO: 141 - protein, 5 aa, Homo sapiens
RDVNY

SEQ ID NO: 142 - protein, 7 aa, Homo sapiens
EKFNLKL